European Patent Specification EP 3 494 223 B1, published February 15, 2023. Title: CONSTRUCTS AND METHODS FOR CONTROLLING STOMATAL CLOSURE IN PLANTS. Applicant: BIOGEMMA COMMISSARIAT A L'ENERGIE ATOMIQUE ET AUX ENERGIES ALTERNATIVES. The sequence listing filed with the application follows.

SEQUENCE LISTING (66 sequences)

SEQ ID NO: 1 - protein, 931 aa, Arabidopsis thaliana
  misc_feature: AtAHA5 wild-type
MEEVFEELKCTKQGLTANEASHRLDVFGPNKLEEKKESKLLKFLGFMWNPLSWVMEVAALMAIALANGGGRPPDWQDFVGIVCLLLINSTISFIEENNAGNAAAALMAGLAPKTKVLRDNQWSEQEASILVPGDVISIKLGDIIPADARLLDGDPLKIDQSSLTGESIPVTKNPSDEVFSGSICKQGEIEAIVIATGVHTFFGKAAHLVDNTNQIGHFQKVLTSIGNFCICSIALGIIVELLVMYPIQRRRYRDGIDNLLVLLIGGIPIAMPSVLSVTMATGSHRLFQQGAITKRMTAIEEMAGMDVLCCDKTGTLTLNKLTVDKNLVEVFAKGVGKEHVFLLAARASRIENQDAIDAAIVGMLADPKEARAGVREVHFFPFNPVDKRTALTYVDSDGNWHRASKGAPEQILNLCNCKEDVRRKVHGVIDKFAERGLRSLAVARQEVLEKKKDAPGGPWQLVGLLPLFDPPRHDSAETIRRALNLGVNVKMITGDQLAIGKETGRRLGMGTNMYPSSALLGQVKDSSLGALPVDELIEKADGFAGVFPEHKYEIVHRLQQRNHICGMTGDGVNDAPALKKADIGIAVVDATDAARGASDIVLTEPGLSVIISAVLTSRAIFQRMKNYTIYAVSITIRIVFGFMFIALIWQFDFSPFMVLIIAILNDGTIMTISKDRMKPSPQPDSWKLRDIFSTGVVLGGYQALMTVVFFWVMKDSDFFSNYFGVRPLSQRPEQMMAALYLQVSIISQALIFVTRSRSWSYAECPGLLLLGAFVIAQLVATFIAVYANWSFARIEGAGWGWAGVIWLYSFLTYIPLDLLKFGIRYVLSGKAWLNLLENKTAFTTKKDYGKEEREAQWAAAQRTLHGLQPAEKNNIFNEKNSYSELSQIAEQAKRRAEVVRLREINTLKGHVESVVKLKGLDIDTIQQHYTV

SEQ ID NO: 2 - protein, 961 aa, Zea mays
  misc_feature: ZmAHA5 wild-type
MGPLQRRPTAMGGLEEIKNEAVDLENIPIEEVFEQLKCTREGLSSSEGQQRLEIFGPNRLEEKKESKILKFLGFMWNPLSWVMEMAAVMAIALANGGGKPPDWEDFVGIIVLLVINSTISFIEENNAGNAAAALMANLAPKTKVLRDGRWGEQEAAILVPGDIVSIKLGDIVPADARLLEGDPLKVDQSALTGESLPVTKGPGDEVFSGSTCKQGEIEAVVIATGVHTFFGKAAHLVDSTNQVGHFQQVLTAIGNFCICSIAVGIVVEIIVMFPIQHRRYRSGIENLLVLLIGGIPIAMPTVLSVTMAIGSHKLSQQGAITKRMTAIEEMAGMDVLCSDKTGTLTLNKLSVDKNLVEVFCKGVDKDHVLLLAARASRTENQDAIDAAMVGMLADPKEARAGIREIHFLPFNPVDKRTALTYIDADGHWHRVSKGAPEQILDLCHCKEDLRRKVHGIIDKYAERGLRSLAVARQEVPERNKESPGGPWQFVGLLPLFDPPRHDSAETIRKALVLGVNVKMITGDQLAIGKETGRRLGMGTNMYPSSALLGQNKDATLEALPVDELIEKADGFAGVFPEHKYEIVKRLQEKKHIVGMTGDGVNDAPALKKADIGIAVADATDAARSASDIVLTEPGLSVIISAVLTSRCIFQRMKNYTIYAVSITIRIVLGFMLIALIWQYDFSPFMVLIIAILNDGTIMTISKDRVKPSPLPDSWKLKEIFATGIVLGSYLALMTVIFFWAMHKTDFFSDKFGVRSIRDSEHEMMSALYLQVSIVSQALIFVTRSRSWSFVERPGLLLVTAFLLAQLVATFLAVYANWGFARIKGIGWGWAGVVWLYSIVFYFPLDLIKFFIRFVLSGRAWDNLLENKTAFTTKKDYGREEREAQWATAQRTLHGLQPPEAATSTLFHDKNSYRELSEIAEQAKRRAEIARLRELNTLKGHVESVVKLKGLDIDTIQQNYTV

SEQ ID NO: 3 - protein, 954 aa, Helianthus annuus
  misc_feature: HaRA11741_4232_Helianthus_annuus
MGTDKALGLEEIKNETVDLEKVPIEEVFQQLKCNREGLTSDEGAARLQIFGPNKLEEKKESKILKFLGFMWNPLSWVMEAAAIMAIAMANGGGKPPDWQDFVGIVCLLVINSTISFIEENNAGNAAAALMAGLAPKTKVLRDGRWSEQEASILVPGDIISIKLGDIVPADARLLEGDPLKIDQSALTGESLPVNKNPYDEVFSGSTCKQGEIEAVVIATGVHTFFGKAAHLVDSTNQVGHFQQVLTAIGNFCICSIAVGMLVEIIVMYPIQHRQYRSGIDNLLVLLIGGIPIAMPTVLSVTMAIGSHRLSQQGAITKRMTAIEEMAGMDVLCSDKTGTLTLNKLTVDKNLIEVFAKGVDKEQVLLYAARASRTENQDAIDAAIVGTLADPKEARAGIREVHFFPFNPVDKRTALTYIDERGNWHRTSKGAPEQILTLCGCKEDMKKKVHAMIDKFAERGLRSLAVGKQEVPEKTKEGPGGPWQFVGLLSLFDPPRHDSAETIRQALHLGVNVKMITGDQLAIAKETGRRLGMGTNMYPSSSLLGDHKDASIATLPIEELIEKADGFAGVFPEHKYEIVKKLQERKHICGMTGDGVNDAPALKKADIGIAVADATDAARSASDIVLTEPGLSVIISAVLTSRAIFQRMKNYTIYAVSITIRIVFGFMFIALIWKFDFSPFMVLIIAILNDGTIMTISKDRVKPSPLPDSWKLKEIFATGIVLGGYLALMTVIFFWIMKDTDFFTEKFGVRSLRNSEVEMMAALYLQVSIVSQALIFVTRSRSWSFIERPGLLLLGAFLAAQLVATLIAVYAEWEFARIKGVGWGWAGVIWLYSIVFYFPLDIMKFAIRYILSGKAWRNMLENKTAFTTKKDYGREEREAQWALAQRTLHGLQAPETSNIFNEKSSYRELSEIAEQAKRRAEVARLREVLTLKGHVESVVKLKGLDIDTIQQHYTV

SEQ ID NO: 4 - protein, 952 aa, Helianthus annuus
  misc_feature: HaRA11742_4232_Helianthus_annuus
MGGDKALSLEEIKNETVDLEKVPIEEVFEQLKCNREGLSSDEGAARLQIFGPNKLEEKKESKLLKFLGFMNPLSWVMEAAAIMAIALANGGGKPPDWQDFVGIVCLLVINSTISFIEENNAGNAAAALMAGLAPKTKVLRDGNWSEQEAAILVPGDIISIKLGDIVPADARLLEGDPLKIDQSALTGESLPVNKNPYDEVFSGSTCKQGIEAVVIATGVHTFFGKAAHLVDSTNQVGHFQQVLTAIGNFCICSIAVGMLVEIVVMYPIQHREYRNGIDNLLVLLIGGIPIAMPTVLSVTMAIGSHRLSQQGAITKRMTAIEEMAGMDVLCSDKTGTLTLNKLSVDKNLIEVFAKGVDKDQVLLYAARASRTENQDAIDAAIVGTLADPKEARAGIREVHFFPFNPVDKRTALTYIDERGNWHRTSKGAPEQILTLCGCKEDMKKKVHAMIDKFAERGLRSLAVAKQEVPEKNKESPGGPWTFIGLLSLFDPPRHDSAETIRRALNLGVNVKMITGDQLAIAKETGRRLGMGTNMYPSSSLLGNHKDASIAAIPIEELIEKADGFAGVFPEHKYEIVKKLQERKHICGMTGDGVNDAPALKKADIGIAVADATDAARGASDIVLTEPGLSVIISAVLTSRAIFQRMKNYTIYAVSITIRIVFGFLFIALIWKFDFSPFMVLIIAILNDGTIMTISKDRVKPSPLPDSWKLKEIFATGIVLGGYLALMTVIFFWIMKDTNFFSDTFGVRSLRHSEVEMMAALYLQVSIVSQALIFVTRSRSWSFIERPGLLLLGAFLAAQLVATLIAVYANWEFARIKGVGWGWAGVIWLYSIVFYFPLDLMKFAIRYILSGKAWNNLLENKTAFTSKKDYGREEREAQWALAQRTLHGLQQPETSNIFNEKSSYRELSEIAEQAKRRAEVARLREVLTLKGHVESVVKLKGLDIDTIQQHYTV

SEQ ID NO: 5 - protein, 952 aa, Lycopersicon esculentum
  misc_feature: LeAHA_XP_004242908.1_Lycopersicon_esculentum
MAKAISLEEIKNETVDLEKIPIEEVFEQLKCSREGLTSDEGANRLQIFGPNKLEEKKESKILKFLGFMWNPLSWVMEMAAIMAIALANGDGKPPDWQDFVGIVCLLVINSTISFIEENNAGNAAAALMAGLAPKTKVLRDGRWSEQEAAILVPGDIISVKLGDIVPADARLLEGDPLKIDQSALTGESLPVTKNPGDEVFSGSTCKQGELEAVVIATGVHTFFGKAAHLVDSTNNVGHFQKVLTAIGNFCICSIAIGMLVEIIVMYPIQHRKYRDGIDNLLVLLIGGIPIAMPTVLSVTMAIGSHRLSQQGAITKRMTAIEEMAGMDVLCSDKTGTLTLNKLSVDRSLVEVFTKGVDKEYVLLLAARASRVENQDAIDACMVGMLADPKEARAGIREVHFLPFNPVDKRTALTYIDSNGNWHRASKGAPEQILDLCNCKEDVRRKVHSMIDKYAERGLRSLAVARQEVPEKSKESTGGPWQFVGLLPLFDPPRHDSAETIRRALNLGVNVKMITGDQLAIAKETGRRLGMGTNMYPSASLLGQDKDSSIASLPVEELIEKADGFAGVFPEHKYEIVKKLQERKHIVGMTGDGVNDAPALKKADIGIAVADATDAARGASDIVLTEPGLSVIISAVLTSRAIFQRMKNYTIYAVSITIRIVFGFMLIALIWKYDFSAFMVLIIAILNDGTIMTISKDRVKPSPMPDSWKLNEIFATGVVLGGYQALMTVIFFWAMHDTSFFTDKFGVKDIRESDEEMMSALYLQVSIISQALIFVTRSRSWSFVERPGALLMIAFLIAQLVATLIAVYADWTFARVKGCGWGWAGVIWIFSIVTYFPLDIMKFAIRYILSGKAWNNLLDNKTAFTTKKDYGKEEREAQWALAQRTLHGLQPPEASNLFNEKNSYRELSEIAEQAKRRAEMARLRELHTLKGHVESVVKLKGLDIETIQQHYTV

SEQ ID NO: 6 - protein, 951 aa, Aeluropus littoralis
  misc_feature: AlAHA_G3M3G8_Aeluropus_littoralis
MGGLEEIKNEAVDLENIPMEEVFEQLKCTREGLSSEEGTQRLQVFGPNKLEEKKESKVLKFLGFMWNPLSWVMEMAAIMAIALANGGGKPPDWQDFVGIIVLLVINSTISFIEENNAGNAAAALMANLAPKTKVLRDGRWGEQEAAILVPGDIISIKLGDIVPADARLLEGDPLKVDQSALTGESLPVTKGPGDEVFSGSTCKQGEIEAVVIATGVHTFFGKAAHLVDSTNQVGHFQQVLTAIGNFCICSIAVGIVIEIIVMFPIQHRKYRSGIENLLVLLIGGIPIAMPTVLSVTMAIGSHKLSQQGAITKRMTAIEEMAGMDVLCSDKTGTLTLNKLSVDKNLVEVFAKGVDKDHVLLLAARASRTENQDAIDAAMVGMLADPKEARAGIREVHFLPFNPVDKRTALTYIDSDGNWHRASKGAPEQIITLCNCREDMKRKVHSIIDKYAERGLRSLAVARQEVPEKTKESPGGPWQFVGLLPLFDPPRHDSAETIRKALHLGVNVKMITGDQLAIGKETGRRLGMGTNMYPSSALLGQNKDSTLEALPVDELIEKADGFAGVFPEHKYEIVKKLQEKKHIVGMTGDGVNDAPALKKADIGIAVADATDAARSASDIVLTEPGLSVIISAVLTSRCIFQRMKNYTIYAVSITIRIVLGFLLIALIWKFDFAPFMVLIIAILNDGTIMTISKDRVKPSPLPDSWKLNEIFATGIVLGTYLAIMTVVFFWAIHKTDFFTEKFGVRSIRDSEHEMMAALYLQVSIVSQALIFVTRSRSWSFVERPGVLLVTAFLLAQLVATLIAVYANWGFARIKGIGWGWAGVVWLYSVVLYFPLDVFKFLIRFALSGRAWDNLLENKTAFTTKKDYGREEREAQWAAAQRTLHGLQPPEVASNTLFNEKSSYRELSEIAEQAKRRAEIARLRELNTLKGHVESVVKLKGLDIDTIQQNYTV

SEQ ID NO: 7 - protein, 951 aa, Aeluropus littoralis
  misc_feature: AlAHA_G9MC80_Aeluropus_littoralis
MGGLEEIKNESVDLENIPMEEVFEQLKCTREGLSSEEGTQRLQVFGPNKLEEKKESKVLKFLGFMWNPLSWVMEMAAIMAIALANGGGKPPDWQDFVGIIVLLVINSTISFIEENNAGNAAAALMANLAPKTKVLRDGRWGEQEAAILVPGDIISIKLGDIVPADARLLEGDPLKVDQSALTGESLPVTKGPGDEVFSGSTCKQGEIEAVVIATGVHTFFGKAAHLVDSTNQVGLFQQVLTAIGNFCICSIAVGIVIEIIVMFPIQHRRYRSGIENLLVLLIGGIPIAMPTVLSVTMAIGSHKLSQQGAITKRMTAIEEMAGMDVLCSDKTGTLTLNKLSVDKNLVEVFAKGVDKDHVLLLAARASRTENQDAIDAAMVGMLADPKEARAGIREVHFLPFNPVDKRTALTYIDSDGNWHRASKGAPEQIITLCNCREDMKRKVHSIIDKYAERGLRSLAVARQEVPEKTKESPGGPWQFVGLLPLFDPPRHDSAETIRKALHLGVNVEMITGDQLAIGKETGRRLGMGTNMYPSSALLGQNKDATLEALPVDELIEKADGFAGVFPEHKYEIVKKLQEKKHIVGMTGDGVNDAPALKKADIGIAVADATDAARGASDIVLTEPGLSVIISAVLTSRCIFQRMKNYTIYAVSITIRIVLGFLLIALIWKFDLAPFMVLIIAILNDGTIMTISKDRVKPSPLPDSWKLKEIFATGIVLGTYLAIMTVVFFWAIHKTDFFTEKFGVRSIRDSEDEMMAALYLQVSIVSQALIFVTRSRSWSFVERPGVLLVTAFLLAQLVATLIAVYADWGFARIKGIGWGWAGVVWLYSVVFYLPLDVFKFLIRFALSGRAWDNLLENKTAFTTKKDYGREEREAQWAAAQRTLHGLQPPEVASNTLFNEKSSYRELSEIAEQAKRRAEIARLRELNTLKGHVESVVKLKGLDIDTIQQNYTV

SEQ ID NO: 8 - protein, 951 aa, Sorghum bicolor
  misc_feature: SbAHA_Sb06g031240_Sorghum_bicolor
MGGLEEIKNEAVDLENIPIEEVFEQLKCTREGLSSSEGQQRLEIFGPNKLEEKKESKILKFLGFMWNPLSWVMEMAAIMAIALANGGGKPPDWEDFVGIIVLLVINSTISFIEENNAGNAAAALMANLAPKTKVLRDGRWGEQEAAILVPGDIISIKLGDIVPADARLLEGDPLKVDQSALTGESLPVTRGPGDEVFSGSTCKQGEIEAVVIATGVHTFFGKAAHLVDSTNQVGHFQQVLTAIGNFCICSIAVGIIVEIIVMFPIQHRKYRSGIENLLVLLIGGIPIAMPTVLSVTMAIGSHKLSQQGAITKRMTAIEEMAGMDVLCSDKTGTLTLNKLSVDKNLVEVFCKGVDKDHVLLLAARASRTENQDAIDAAMVGMLADPKEARAGIREVHFLPFNPVDKRTALTYIDGDGNWHRVSKGAPEQILDLCHCKEDLRRKVHGIIDKYAERGLRSLAVARQEVPEKNKESPGGPWQFVGLLPLFDPPRHDSAETIRKALVLGVNVKMITGDQLAIGKETGRRLGMGTNMYPSSALLGQNKDSTLEALPVDELIEKADGFAGVFPEHKYEIVKRLQEKKHIVGMTGDGVNDAPALKKADIGIAVADATDAARSASDIVLTEPGLSVIISAVLTSRCIFQRMKNYTIYAVSITIRIVLGFMLIALIWKYDFSPFMVLIIAILNDGTIMTISKDRVKPSPLPDSWKLKEIFATGIVLGSYLAIMTVIFFWAMHKTDFFSDKFGVRSIRDSEHEMMSALYLQVSIVSQALIFVTRSRSWSFVERPGLLLVTAFLLAQLVATFLAVYANWGFARIKGIGWGWAGVVWLYSIVFYFPLDLIKFFIRFVLSGRAWDNLLENKTAFTTKKDYGREEREAQWATAQRTLHGLQPPEAATNTLFNDKSSYRELSEIAEQAKRRAEIARLRELNTLKGHVESVVKLKGLDIDTIQQNYTV

SEQ ID NO: 9 - protein, 951 aa, Setaria italica
  misc_feature: SiAHA_K3Z3J5_Setaria_italica
MGGLEEIKNEAVDLENIPIEEVFEQLKCTREGLSSNEGAQRLEIFGPNKLEEKKESKILKFLGFMWNPLSWVMEMAAIMAIALANGGGKPPDWEDFVGIIVLLVINSTISFIEENNAGNAAAALMANLAPKTKVLRDGRWGEQEAAILVPGDIISIKLGDIVPADARLLEGDPLKVDQSALTGESLPVTKGPGDEVFSGSTCKQGEIEAVVIATGVHTFFGKAAHLVDSTNQVGHFQKVLTAIGNFCICSIAVGIVIEIIVMFPIQHRAYRSGIENLLVLLIGGIPIAMPTVLSVTMAIGSHKLSQQGAITKRMTAIEEMAGMDVLCSDKTGTLTLNKLSVDKNLVEVFCKGVDKDHVLLLAARASRTENQDAIDAAMVGMLADPKEARAGIREVHFLPFNPVDKRTALTYIDSDGNWHRVSKGAPEQILDLCNCREDMRRKVHSIIDKYAERGLRSLAVARQEVPEKSKDASGGPWQFVGLLPLFDPPRHDSAETIRKALVLGVNVKMITGDQLAIGKETGRRLGMGTNMYPSSSLLGTNKDSTLESLPVDELIEKADGFAGVFPEHKYEIVKRLQEKKHIVGMTGDGVNDAPALKKADIGIAVADATDAARSASDIVLTEPGLSVIISAVLTSRCIFQRMKNYTIYAVSITIRIVLGFMLIALIWKYDFSPFMVLIIAILNDGTIMTISKDRVKPSPLPDSWKLKEIFATGVVLGSYLALMTVIFFWAMHKTDFFPEKFGVKPIRDSEGKMMSALYLQVSIVSQALIFVTRSRSWSFVERPGLLLVTAFLLAQLVATFLAVYANWGFARIEGIGWGWAGVVWLYSIVFYFPLDLFKFFIRFVLSGRAWDNLLENKTAFTTKKDYGREEREAQWATAQRTLHGLQPPEAASNTLFNDKSSYRELSEIAEQAKRRAEIARLRELNTLKGHVESVVKLKGLDIDTIQQNYTV

SEQ ID NO: 10 - protein, 951 aa, Oryza sativa
  misc_feature: Os04g56160_Oryza_sativa
MGGLEEIKNEAVDLENIPIEEVFEQLKCTREGLSSEEGNRRIEMFGPNKLEEKKESKILKFLGFMWNPLSWVMEMAAIMAIALANGGGKPPDWEDFVGIIVLLVINSTISFIEENNAGNAAAALMANLAPKTKVLRDGRWGEQEAAILVPGDIISIKLGDIVPADARLLEGDPLKIDQSALTGESLPVTKNPGDEVFSGSTCKQGEIEAVVIATGVHTFFGKAAHLVDSTNQVGHFQTVLTAIGNFCICSIAVGIVIEIIVMFPIQHRAYRSGIENLLVLLIGGIPIAMPTVLSVTMAIGSHKLSQQGAITKRMTAIEEMAGMDVLCSDKTGTLTLNKLSVDKNLVEVFTKGVDKDHVLLLAARASRTENQDAIDAAMVGMLADPKEARAGIREVHFLPFNPVDKRTALTYIDADGNWHRASKGAPEQILTLCNCKEDVKRKVHAVIDKYAERGLRSLAVARQEVPEKSKESAGGPWQFVGLLPLFDPPRHDSAETIRKALHLGVNVKMITGDQLAIGKETGRRLGMGTNMYPSSALLGQNKDASLEALPVDELIEKADGFAGVFPEHKYEIVKRLQEKKHIVGMTGDGVNDAPALKKADIGIAVADATDAARSASDIVLTEPGLSVIISAVLTSRCIFQRMKNYTIYAVSITIRIVLGFLLIALIWKYDFSPFMVLIIAILNDGTIMTISKDRVKPSPLPDSWKLKEIFATGIVLGSYLALMTVIFFWAMHKTDFFTDKFGVRSIRNSEHEMMSALYLQVSIVSQALIFVTRSRSWSFIERPGLLLVTAFMLAQLVATFLAVYANWGFARIKGIGWGWAGVIWLYSIVFYFPLDIFKFFIRFVLSGRAWDNLLENKIAFTTKKDYGREEREAQWATAQRTLHGLQPPEVASNTLFNDKSSYRELSEIAEQAKRRAEIARLRELNTLKGHVESVVKLKGLDIDTIQQNYTV

SEQ ID NO: 11 - protein, 951 aa, Brachypodium distachyon
  misc_feature: BdAHA_Bradi5g24690.1_Brachypodium_distachyon
MGGLEEIRNEAVDLENIPIEEVFEQLKCTREGLTSDEGAQRVTIFGLNKLEEKKESKVLKFLGFMWNPLSWVMEMAAIMAIALANGEGKPPDWQDFVGIIVLLVINSTISFIEENNAGNAAAALMANLAPKTKVLRDGRWGEQEASILVPGDIVSIKLGDIVPADARLLEGDPLKIDQSGLTGESLPVTKNPGDEVFSGSTCKQGEIEAVVIATGVHTFFGKAAHLVDSTNQVGHFQKVLTAIGNFCIVSIAVGIVIEIIVMFPIQRRKYRAGIENLLVLLIGGIPIAMPTVLSVTMAIGSHKLSQQGAITKRMTAIEELAGMDVLCSDKTGTLTLNKLSVDKNLVEVFAKGVDKEHVLLLAARASRVENQDAIDACMVGMLADPKEARAGIREVHFLPFNPTDKRTALTYIDAEGNWHRASKGAPEQIITLCNCKEDVKRKVHSVIEKYAERGLRSLAVARQEVPEKSKDSPGGPWQFIGLLPLFDPPRHDSAETIRKALVLGVNVKMITGDQLAIGKETGRRLGMGTNMYPSSALLGQSKDGSLESLPVDELIEKADGFAGVFPEHKYEIVKRLQEKKHIVGMTGDGVNDAPALKKADIGIAVDDATDAARSASDIVLTEPGLSVIISAVLTSRCIFQRMKNYTIYAVSITIRIVLGFMLIALIWKFDFAPFMVLIIAILNDGTIMTISKDRVKPSPLPDSWKLNEIFATGVVLGTYLALMTVVFFWAIHKTDFFTNKFGVRSIRNSEFELMSALYLQVSIVSQALIFVTRSRSWSFVERPGFLLVTAFLLAQLVATLIAVYANWEFARIKGIGWGWAGVIWLFSIVFYFPLDVFKFFIRFVLSGRAWDNLLQNKTAFTTKKDYGRGEREAQWATAQRTLHGLQAPESNNNTLFNDKSSYRELSEIAEQAKRRAEIARLRELNTLKGHVESVVKLKGLDIDTINQNYTV

SEQ ID NO: 12 - protein, 951 aa, Hordeum vulgare
  misc_feature: HvAHA_M0Z2H5_Hordeum_vulgare
MGGLEEIRNEAVDLENIPIEEVFEQLKCTRQGLTSDEGAQRVEIFGLNKLEEKKESKVLKFLGFMWNPLSWVMEMAAIMAIALANGGGKPPDWQDFVGIIVLLVINSTISFIEENNAGNAAAALMANLAPKTKVLRDGRWGEQEASILVPGDIVSIKLGDIVPADARLLEGDPLKIDQSGLTGESLPVTKNPGDEVFSGSTCKQGEIEAVVIATGVHTFFGKAAHLVDSTNQVGHFQQVLTAIGNFCIISIAVGIVIEIIVMFPIQRRKYRAGIENLLVLLIGGIPIAMPTVLSVTMAIGSHKLSQQGAITKRMTAIEELAGMDVLCSDKTGTLTLNKLSVDKNLVEVFAKGVDKEHVLLLAARASRVENQDAIDACMVGMLADPKEARAGIREVHFLPFNPTDKRTALTYIDAEGNWHRASKGAPEQIITLCNCKEDVKRKVHSVIEKYAERGLRSLAVARQEVPEKSKDSAGGPWQFIGLLPLFDPPRHDSAETIRKALVLGVNVKMITGDQLAIGKETGRRLGMGTNMYPSSALLGQSKDGSLESLPVDELIEKADGFAGVFPEHKYEIVKRLQEKKHIVGMTGDGVNDAPALKKADIGIAVDDATDAARSASDIVLTEPGLSVIISAVLTSRCIFQRMKNYTIYAVSITIRIVLGFLLIALIWKFDFAPFMVLIIAILNDGTIMTISKDRVKPSPLPDSWKLNEIFATGVVLGTYLALMTVVFFWIIHRTDFFTNKFGVRSIRENETEKMSALYLQVSIVSQALIFVTRSRSWSFVERPGFLLVIAFLLAQLVATLIAVYANWGFARISGIGWGWAGVIWLFSIVFYFPLDIFKFFIRFVLSGRAWDNLLQNKTAFTTKENYGKGEREAQWATAQRTLHGLQAPEPASHTLFNDKSSYRELSEIAEQAKRRAEIARLRELNTLKGHVESVVKLKGLDIDTINQNYTV

SEQ ID NO: 13 - protein, 956 aa, Hordeum vulgare
  misc_feature: HvAHA_Q8H1X2_Hordeum_vulgare
MADKEAGNLEAVLKEVVDLENIPLEEVLDNLRCSREGLTAEQAQQRLQILGPNKLEEKEESKFLKFLGFMWNPLSWVMEMAAIMAIALANGGGKPPDWQDFVGIIVLLVINSTVSFIEENNAGNAAAALMANLAPKTKVLRDGRWGEQEASILVPGTLSASSLVTSSLLMLVCLEGDPFEDSSVWAYRRVSPSDQEPWGEVFSGSTCKQGEIEAVVIATGVHTFFGKAAHLVDSTNQVGHFQQVLTAIGNFCIISIAVGIVIEIIVMFPIQRRKYRAGIENLLVLLIGGIPIAMPTVLSVTMAIGSHKLSQQGAITKRMTAIEELAGMDVLCSDKTGTLTLNKLSVDKNLVEVFAKGVDKEHVLLLAARASRVENQDAIDACMVGMLADPKEARAGIREVHFLPFNPTDKRTALTYIDAEGNWHRASKGAPEQIITLCNCKEDVKRKVHSVIEKYAERGLRSLAVARQEVPEKSKDSAGGPWQFIGLLPLFDPPRHDSAETIRKALVLGVNVKMITGDQLAIGKETGRRLGMGTNMYPSSALLGQSKDGSLESLPVDELIEKADGFAGVFPEHKYEIVKRLQEKKHIVGMTGDGVNDAPALKKADIGIAVDDATDAARSASDIVLTEPGLSVIISAVLTSRCIFQRMKNYTIYAVSITIRIVLGFLLIALIWKFDFAPFMVLIIAILNDGTIMTISKDRVKPSPLPDSWKLNEIFATGVVLGTYLALMTVVFFWIIHRTDFFTNKFGVRSIRENETEKMSALYLQVSIVSQALIFVTRSRSWSFVERPGFLLVIAFLLAQLVATLIAVYANWGFARISGIGWGWAGVIWLFSIVFYFPLDIFKFFIRFVLSGRAWDNLLQNKTAFTTKENYGKGEREAQWATAQRTLHGLQAPEPASHTLFNDKSSYRELSEIAEQAKRRAEIARLRELNTLKGHVESVVKLKGLDIDTINQNYTV

SEQ ID NO: 14 - protein, 880 aa, Triticum aestivum
  misc_feature: TaAHA_2BL_4AEA2109C_Triticum_aestivum
MWNPLSWVMEMAAIMAIALANGGGKPPDWQDFVGIIVLLVINSTISFIEENNAGNAAAALMANLAPKTKVLRDGRWGEQEASILVPGDIVSIKLGDIVPADARLLEGDPLKIDQSGLTGESLPVTKNPGDEVFSGSTCKQGEIEAVVIATGVHTFFGKAAHLVDSTNQVGHFQQVLTAIGNFCIVSIAVGIVIEIIVMFPIQRRKYRAGIENLLVLLIGGIPIAMPTVLSVTMAIGSHKLSQQGAITKRMTAIEELAGMDVLCSDKTGTLTLNKLSVDKNLVEVFAKGVDKEHVLLLAARASRVENQDAIDACMVGMLADPKEARAGIREVHFLPFNPTDKRTALTYIDAEGNWHRASKGAPEQIITLCNCKEDVKRKVHSVIEKYAERGLRSLAVARQEVPEKSKDSPGGPWQFIGLLPLFDPPRHDSAETIRKALVLGVNVKMITGDQLAIGKETGRRLGMGTNMYPSSALLGQSKDGSLESLPVDELIEKADGFAGVFPEHKYEIVKRLQEKKHIVGMTGDGVNDAPALKKADIGIAVDDATDAARSASDIVLTEPGLSVIISAVLTSRCIFQRMKNYTIYAVSITIRIVLGFMLIALIWKFDFAPFMVLIIAILNDGTIMTISKDRVKPSPLPDSWKLNEIFATGVVLGTYLALMTVVFFWVIHKTDFFTNKFGVRSIRDSEFEMMSALYLQVSIVSQALIFVTRSRSWSFVERPGFLLVTAFLLAQLVATLIAVYANWEFARIKGIGWGWAGVIWLFSIVFYFPLDIFKFFIRFVLSGRAWDNLLQNKTAFTTKENYGKGEREAQWATAQRTLHGLQAPEPASHTLFNDKSSYRELSEIAEQAKRRAEIARLRELNTLKGHVESVVKLKGLDIDT

SEQ ID NO: 15 - protein, 951 aa, Triticum aestivum
  misc_feature: TaAHA_2AL_2C50DEE4C.1_Triticum_aestivum
MGGLEEIRNEAVDLENIPIEEVFEQLKCTRQGLTSDEGAQRVEIFGLNKLEEKKESKVLKFLGFMWNPLSWVMEMAAIMAIALANGGGKPPDWQDFVGIIVLLVINSTISFIEENNAGNAAAALMANLAPKTKVLRDGRWGEQEASILVPGDIVSIKLGDIVPADARLLEGDPLKIDQSGLTGESLPVTKNPGDEVFSGSTCKQGEIEAVVIATGVHTFFGKAAHLVDSTNQVGHFQQVLTAIGNFCIVSIAVGIVIEIIVMFPIQRRKYRAGIENLLVLLIGGIPIAMPTVLSVTMAIGSHKLSQQGAITKRMTAIEELAGMDVLCSDKTGTLTLNKLSVDKNLVEVFAKGVDKEHVLLLAARASRVENQDAIDACMVGMLADPKEARAGIREVHFLPFNPTDKRTALTYIDAEGNWHRASKGAPEQIITLCNCKEDVKRKVHSVIEKYAERGLRSLAVARQEVPEKSKDSPGGPWQFIGLLPLFDPPRHDSAETIRKALVLGVNVKMITGDQLAIGKETGRRLGMGTNMYPSSALLGQSKDGSLESLPVDELIEKADGFAGVFPEHKYEIVKRLQEKKHIVGMTGDGVNDAPALKKADIGIAVDDATDAARSASDIVLTEPGLSVIISAVLTSRCIFQRMKNYTIYAVSITIRIVLGFMLIALIWKFDFAPFMVLIIAILNDGTIMTISKDRVKPSPLPDSWKLNEIFATGVVLGTYLALVTVVFFWLIHKTDFFTNKFGVESIRNTEFKEMSALYLQVSIVSQALIFVTRSRSWSFVERPGFLLVTAFLLAQLVATLIAVYANWDFARIKGIGWGWAGVIWLFSIVFYFPLDIFKFFIRFVLSGRAWDNLLQNKTAFTTKENYGKGEREAQWATAQRTLHGLQAPEPASHTLFNDKSSYRELSEIAEQAKRRAEIARLRELNTLKGHVESVVKLKGLDIDTINQNYTV

SEQ ID NO: 16 - protein, 951 aa, Triticum aestivum
  misc_feature: TaAHA_Q5PSM6_Triticum_aestivum
MGGLEEIRNEAVDLENIPIEEVFEQLKCTRQGLTSDEGAQRVEIFGLNKLEEKKESKVLKFLGFMWNPLSWVMEMAAIMAIALANGGGKPPDWQDFVGIIVLLVINSTISFIEENNAGNAAAALMANLAPKTKVLRDGRWGEQGASILVPGDIVSIKLGDIVPADARLLEGDPLKIDQSGLTGESLPVTKNPGDEVFSGSTCKQGEIEAVVIATGVRTFFGKAAHLVDSTNQVGHFQQVLTAIGNFCIVSIAVGIVIEIIVMFPIQRRKYRAGIENLLVLLIGGIPIAMPTVLSVTMAIGSHKLSQQGAITKRMTAIEELAGMDVLCSDKTGTLTLNKLSVDKNLVEVFAKGVDKEHVLLLAARASRVENQDAIDACMVGMLADPKEARAGIREVHFLPFNPTDKRTALTYIDAEGNWHRASKGAPEQIITLCNCKEDVKRKVHSVIEKYAERGLRSLAVARQEVPEKSKDSPGGPWQFIGLLPLFDPPRHDSAETIRKALVLGVNVKMITGDQLAIGKETGRRLGMGTNMYPSSALLGQSKDGSLESLPVDELIEKADGFAGVFPEHKYEIVKRLQEKKHIVGMTGDGVNDAPALKKADIGIAVDDATDAARSASDIVLTEPGLSVIISAVLTSRCIFQRMKNYTIYAVSITIRIVLGFMLIALIWKFDFAPFMVLIIAILNDGTIMTISKDRVKPSPLPDSWKLNEIFATGVVLGTYLALVTVVFFWLIHKTDFFTNKFGVESIRNTEFKEMSALYLQVSIVSQALIFVTRSRSWSFVERPGFLLVTAFLLAQLVATLIAVYANWDFARIKGIGWGWAGVIWLFSIVFYFPLDIFKFFIRFVLSGRAWDNLLQNKTAFTTKENYGKGEREAQWATAQRTLHGLQAPEPASHTLFNDKSSYRELSEIAEQAKRRAEIARLRELNTLKSHVESVVKLKGLDIDTINQNYTV

SEQ ID NO: 17 - protein, 931 aa, Capsella rubella
  misc_feature: CrAHA|XP_006293643_Capsella_rubella
MEEVFEELKCTKQGLTREEASHRLDLFGPNKLEEKKESKVLKFLGFMWNPLSWVMEAAALMAIALANGGGRPPDWQDFVGIVCLLFINSTISFIEENNAGNAAAALMAGLAPKTKVLRDNQWSEQEASILVPGDVISVKLGDIIPADARLLDGDPLKIDQSSLTGESIPVTKNPGDEVFSGSTCKQGEIEAIVVATGVHTFFGKAAHLVDSTNQIGHFQKVLTSIGNFCICSIGLGIIVELIVMYPIQRRKYRDGIDNLLVLLIGGIPIAMPTVLSVTMAIGSHRLSKQGAITKRMTAIEEMAGMDVLCSDKTGTLTLNRLTVDRNLVEVFAKGVGKEHVFLLAARASRIENQDAIDAAIVGMLGDPKEARAGVREVHFFPFNPVDKRTALTYIDSDGNWHRASKGAPEQILNLCNCKEDVRRKVHGVIDKFAERGLRSLAVARQKVPEKKKDASGDPWQLVGLLPLFDPPRHDSAETIRRALNLGVNVKMITGDQLAIGKETGRRLGMGTNMYPSSALLGQEKDSSLGALPVDELIEKADGFAGVFPEHKYEIVNRLQQRKHICGMTGDGVNDAPALKKADIGIAVADATDAARGASDIVLTEPGLSVIISAVLTSRAIFQRMKNYTIYAVSITIRIVFGFMFIALIWQFDFSPFMVLIIAILNDGTIMTISKDRVKPSPQPDSWKLREIFSTGVVLGGYQALMTVVFFWVMKDTDIFSNMLGVRPLSQRPEQMMAALYLQVSIISQALIFVTRSRSWSFVERPGLLLLGAFVIAQLVATFIAVYANWSFARIEGAGWGWAGVIWLYSLITYIPLDLLKFGIRYVLSGKAWLNLLENKTAFTTKKDYGKEEREAQWAAAQRTLHGLQPAETNNIFNEKNSYHDLSQIAEQAKRRAEVVRLREINTLKGHVESVVKLKGLDIDTIQQHYTV

SEQ ID NO: 18 - protein, 957 aa, Camelina sativa
  misc_feature: CsAHA|XP_010472461_Camelina_sativa
MAAAAGKGNELDHIKNESVDLVRIPMEEVFEELKCTKQGLTTDEASHRLDLFGPNKLEEKKESKLLKFLGFMWNPLSWVMEAAALMAIALANGGGRPPDWQDFVGIVCLLFINSTISFIEENNAGNAAAALMAGLAPKTKVLRDNQWSEQEASILVPGDVISLKLGDIIPADARLLDGDPLKIDQSSLTGESIPVTKNPGDEVFSGSTCKQGEIEAIVVATGVHTFFGKAAHLVDSTNQIGHFQKVLTSIGNFCICSIALGIVVELLVMYPIQRRGYRDGIDNLLVLLIGGIPIAMPTVLSVTMAIGSHRLSKQGAITKRMTAIEEMAGMDVLCSDKTGTLTLNKLTVDRNLVEVFAKGVGKEHVFLLAARASRIENQDAIDAAIVGMLADPKEARAGVREVHFFPFNPVDKRTALTYVDYSDGNWYRASKGAPEQILNLCDCKEDVRRKVHGVIDKFAERGLRSLAVARQEVPEKKKDASGGPWQLVGLLPLFDPPRHDSAETIRRALNLGVNVKMITGDQLAIGKETGRRLGMGTNMYPSSALLGQEKDSSLGALPVDELIEKADGFAGVFPEHKYEIVNRLQQRKHICGMTGDGVNDAPALKKADIGIAVADSTDAARGASDIVLTEPGLSVIISAVLTSRAIFQRMKNYTIYAVSITIRIVFGFMFIALIWQFDFSPFMVLIIAILNDGTIMTISKDRVKPSPQPDSWKLREIFSTGVVLGGYQAFMTVVFFWVMKDTNIFSNMLGVRPLSQRPEQMMAALYLQVSIISQALIFVTRSRSWSFVERPGLLLLGAFVIAQLVATFIAVYADWSFARIEGAGWGWAGVIWLYSLITYIPLDLLKFGIRYVLSGKAWLNLLENKTAFTTKKDYGKEEREAQWAAAQRTLHGLQPAETNNIFNEKNSYSELSQIAEQAKRRAEVVRLREINSLKGHVESVVKLKGLDIDTIQQHYTV

SEQ ID NO: 19 - protein, 951 aa, Medicago truncatula
  misc_feature: MtAHA|XP_013465721_Medicago_truncatula
MGGISLEEIKNESVDLERIPIDEVFEQLKCSRQGLTSEEGANRLQVFGPNKLEEKKESKFLKFLGFMWNPLSWVMEAAAIMAIALANGSGRPPDWQDFVGIIALLVINSTISFIEENNAGNAAAALMAGLAPKTKVLRDSRWSEQDAAILVPGDIISIKLGDIVPADARLLEGDPLSIDQSALTGESLPVTKSSSDEVFSGSTVKKGEIEAVVIATGVHTFFGKAAHLVDSTNQVGHFQKVLTAIGNFCICSIAIGILVELIVMYPIQHRKYRDGIDNLLVLLIGGIPIAMPTVLSVTMAIGSHRLSQQGAITKRMTAIEEMAGMDVLCSDKTGTLTLNKLSVDRNLIEVFAKGIEKEYVMLLAARASRTENQDAIDAAIVGMLADPKEARAGIREVHFLPFNPVDKRTALTYIDSDGKWHRASKGAPEQIINLCNCKEDVRKKVHAVIDKFAERGLRSLGVARQEVPERTKDSPGGPWQFVGLLPLFDPPRHDSAETIRRALNLGVNVKMITGDQLAIGKETGRRLGMGTNMYPSSALLGQDKDSSISALPVDELIEKADGFAGVFPEHKYEIVKRLQEKKHICGMTGDGVNDAPALKKADIGIAVADATDAARSASDIVLTEPGLSVIISAVLTSRAIFQRMKNYTIYAVSITIRIVFGFMFIALIWKFDFAPFMVLIIAILNDGTIMTISKDRVKPSPLPDSWKLREIFATGVVLGSYMALMTVVFFWAMKDTNFFSNKFGVRPIRHNPDEMMAALYLQVSIISQALIFVTRSRSWSFAERPGLLLLGAFLIAQLIATFIAVYANWGFARIKGMGWGWAGVIWLYSLVTYIPLDLLKFAIRYFLSGKAWDNLLENKTAFTTKKDYGKEEREAQWAAAQRTLHGLQPPEASNVFNEKNSYRELSEIAEQAKRRAEVARLREVHTLKGHVESVVKLKGLDIDTIQQHYTV

SEQ ID NO: 20 - protein, 955 aa, Populus euphratica
  misc_feature: PeAHA|XP_011031360_Populus_euphratica
MSSKGGISLEEIKNESVDLERIPMEEVFEQLKCTREGLSADEGASRLQVFGPNKLEEKKESKILKFLGFMWNPLSWVMEAAALMAIALANGDGRPPDWQDFVGIVVLLVINSTISFIEENNAGNAAAALMAGLAPKTKVLRDGRWSEQDASILVPGDIISIKLGDIVPADARLLEGDPLKIDQSALTGESLPVTKNPSDEVFSGSTCKQGEIEAVVIATGVHTFFGKAAHLVDSTNQVGHFQKVLTAIGNFCICSIAVGIFAELIVMYPIQHRKYRDGIDNLLVLLIGGIPIAMPTVLSVTMAIGSHRLSQQGAITKRMTAIEEMAGMDVLCSDKTGTLTLNKLTVDRSLIEVFAKGVEKEHVILLAARASRTENQDAIDAAIVGMLADPKEARAGIREVHFLPFNPVDKRTALTYIDSDGNWHRASKGAPEQILTLCNCKEDVKKKVHSVIDKFAERGLRSLGVAKQEVPEKSKDAAGAPWQLVGLLPLFDPPRHDSAETIRRALHLGVNVKMITGDQLAIGKETGRRLGMGTNMYPSSALLGQDRDASIAALPVDELIEKADGFAGVFPEHKYEIVKRLQDRKHICGMTGDGVNDAPALKKADIGIAVADATDAARSASDIVLTEPGLSVIISAVLTSRAIFQRMKNYTIYAVSITIRIVFGFMFIALIWKFDFAPFMVLIIAILNDGTIMTISKDRVKPSPQPDSWKLKEIFSTGIVLGGYMALMTVLFFWIMKDTDFFSDKFGVRSLRKNDEEMMAALYLQVSIVSQALIFVTRSRSWSFVERPGFLLLGAFVAAQLIATLIAVYANWGFARIKGCGWGWAGVIWLFSVVTYVPLDILKFAIRYILSGKAWDNLLENKTAFTTKKDYGKEEREAQWATAQRTLHGLQPPETSHNMFSEKNSYRELSEIAEQAKRRAEMARLRELNTLKGHVESVVKLKGLDIDTIQQHYTV

SEQ ID NO: 21 - protein, 23 aa, Artificial
  Consensus sequence First transmembrane domain
  VARIANT (15)..(15): Xaa can be replaced by  M, V, A
  VARIANT (18)..(18): Xaa can be replaced by  L, I, V
  VARIANT (23)..(23): Xaa can be replaced by  L, M
FLGFMWNPLSWVMEXAAXMAIAX

SEQ ID NO: 22 - protein, 23 aa, Artificial
  First transmembrane domain mutated at position 8 P->S
  VARIANT (15)..(15): Xaa can be replaced by  M, V, A
  VARIANT (18)..(18): Xaa can be replaced by  L, I, V
  VARIANT (23)..(23): Xaa can be replaced by  L, M
FLGFMWNSLSWVMEXAAXMAIAX

SEQ ID NO: 23 - protein, 930 aa, Arabidopsis thaliana
  misc_feature: AtAHA5_P50S mutant
MEEVFEELKCTKQGLTANEASHRLDVFGPNKLEEKKESKLLKFLGFMWNSLSWVMEVAALMAIALANGGGRPPDWQDFVGIVCLLLINSTISFIEENNAGNAAAALMAGLAPKTKVLRDNQWSEQEASILVPGDVISIKLGDIIPADARLLDGDPLKIDQSSLTGESIPVTKNPSDEVFSGSICKQGEIEAIVIATGVHTFFGKAAHLVDNTNQIGHFQKVLTSIGNFCICSIALGIIVELLVMYPIQRRRYRDGIDNLLVLLIGGIPIAMPSVLSVTMATGSHRLFQQGAITKRMTAIEEMAGMDVLCCDKTGTLTLNKLTVDKNLVEVFAKGVGKEHVFLLAARASRIENQDAIDAAIVGMLADPKEARAGVREVHFFPFNPVDKRTALTYVDSDGNWHRASKGAPEQILNLCNCKEDVRRKVHGVIDKFAERGLRSLAVARQEVLEKKKDAPGGPWQLVGLLPLFDPPRHDSAETIRRALNLGVNVKMITGDQLAIGKETGRRLGMGTNMYPSSALLGQVKDSSLGALPVDELIEKADGFAGVFPEHKYEIVHRLQQRNHICGMTGDGVNDAPALKKADIGIAVVDATDAARGASDIVLTEPGLSVIISAVLTSRAIFQRMKNYTIYAVSITIRIVFGFMFIALIWQFDFSPFMVLIIAILNDGTIMTISKDRMKPSPQPDSWKLRDIFSTGVVLGGYQALMTVVFFWVMKDSDFFSNYFGVRPLSQRPEQMMAALYLQVSIISQALIFVTRSRSWSYAECPGLLLLGAFVIAQLVATFIAVYANWSFARIEGAGWGWAGVIWLYSFLTYIPLDLLKFGIRYVLSGKAWLNLLENKTAFTTKKDYGKEEREAQWAAAQRTLHGLQPAEKNNIFNEKNSYSELSQIAEQAKRRAEVVRLREINTLKGHVESVVKLKGLDIDTIQQHYT

SEQ ID NO: 24 - protein, 107 aa, Artificial
  Consensus sequence R1 domain
  VARIANT (4)..(4): Xaa can be replaced by  R, K
  VARIANT (7)..(7): Xaa can be replaced by  D, L, N, R
  VARIANT (9)..(9): Xaa can be replaced by  L, M
  VARIANT (11)..(11): Xaa can be replaced by  E, Q, D
  VARIANT (14)..(14): Xaa can be replaced by  T, I
  VARIANT (18)..(18): Xaa can be replaced by  T, S
  VARIANT (20)..(20): Xaa can be replaced by  K, E
  VARIANT (21)..(21): Xaa can be replaced by  D, N
  VARIANT (24)..(24): Xaa can be replaced by  K, R
  VARIANT (25)..(25): Xaa can be replaced by  E, G
  VARIANT (33)..(33): Xaa can be replaced by  T, A, L
  VARIANT (43)..(43): Xaa can be replaced by  P, A
  VARIANT (44)..(44): Xaa can be replaced by  P, A
  VARIANT (46)..(46): Xaa can be replaced by  T, V, A, P, K, S
  VARIANT (47)..(47): Xaa can be replaced by A, S, N
  VARIANT (48)..(48): Xaa can be replaced by S, T, N
  VARIANT (49)..(49): Xaa can be replaced by  N, S, H
  VARIANT (50)..(50): Xaa can be replaced by  N, T
  VARIANT (51)..(51): Xaa can be replaced by  I, V, M, L
  VARIANT (53)..(53): Xaa can be replaced by  N, S, H
  VARIANT (54)..(54): Xaa can be replaced by  E, D
  VARIANT (56)..(56): Xaa can be replaced by  S, N
  VARIANT (59)..(59): Xaa can be replaced by  R, S, H
  VARIANT (60)..(60): Xaa can be replaced by  E, D
  VARIANT (63)..(63): Xaa can be replaced by  E, Q
  VARIANT (74)..(74): Xaa can be replaced by  I, V, M
  VARIANT (75)..(75): Xaa can be replaced by  A, V
  VARIANT (80)..(80): Xaa can be replaced by  L, I, V
  VARIANT (81)..(81): Xaa can be replaced by  N, L, H
  VARIANT (82)..(82): Xaa can be replaced by  T, S
  VARIANT (85)..(85): Xaa can be replaced by  G, S
  VARIANT (99)..(99): Xaa can be replaced by  D, E
  VARIANT (102)..(102): Xaa can be replaced by  Q, N
  VARIANT (104)..(104): Xaa can be replaced by  N, H
LSGXAWXNXLXNKXAFTXKXXYGXXEREAQWAXAQRTLHGLQXXEXXXXXXFXXKXSYXXLSXIAEQAKRRAEXXRLREXXXLKXHVESVVKLKGLDIXTIXQXYTV

SEQ ID NO: 25 - protein, 106 aa, Artificial
  Consensus sequence R1 domain
  VARIANT (4)..(4): Xaa can be replaced by  R, K
  VARIANT (7)..(7): Xaa can be replaced by  D, L, N, R
  VARIANT (9)..(9): Xaa can be replaced by  L, M
  VARIANT (11)..(11): Xaa can be replaced by  E, Q, D
  VARIANT (14)..(14): Xaa can be replaced by  T, I
  VARIANT (18)..(18): Xaa can be replaced by  T, S
  VARIANT (20)..(20): Xaa can be replaced by  K, E
  VARIANT (21)..(21): Xaa can be replaced by  D, N
  VARIANT (24)..(24): Xaa can be replaced by  K, R
  VARIANT (25)..(25): Xaa can be replaced by  E, G
  VARIANT (33)..(33): Xaa can be replaced by  T, A, L
  VARIANT (43)..(43): Xaa can be replaced by  P, A
  VARIANT (44)..(44): Xaa can be replaced by  P, A
  VARIANT (46)..(46): Xaa can be replaced by  T, V, A, P, K, S
  VARIANT (47)..(47): Xaa can be replaced by S, T, N
  VARIANT (48)..(48): Xaa can be replaced by  N, S, H
  VARIANT (49)..(49): Xaa can be replaced by  N, T
  VARIANT (50)..(50): Xaa can be replaced by  I, V, M, L
  VARIANT (52)..(52): Xaa can be replaced by  N, S, H
  VARIANT (53)..(53): Xaa can be replaced by  E, D
  VARIANT (55)..(55): Xaa can be replaced by  S, N
  VARIANT (58)..(58): Xaa can be replaced by  R, S, H
  VARIANT (59)..(59): Xaa can be replaced by  E, D
  VARIANT (62)..(62): Xaa can be replaced by  E, Q
  VARIANT (73)..(73): Xaa can be replaced by  I, V, M
  VARIANT (74)..(74): Xaa can be replaced by  A, V
  VARIANT (79)..(79): Xaa can be replaced by  L, I, V
  VARIANT (80)..(80): Xaa can be replaced by  N, L, H
  VARIANT (81)..(81): Xaa can be replaced by  T, S
  VARIANT (84)..(84): Xaa can be replaced by  G, S
  VARIANT (98)..(98): Xaa can be replaced by  D, E
  VARIANT (101)..(101): Xaa can be replaced by  Q, N
  VARIANT (103)..(103): Xaa can be replaced by  N, H
LSGXAWXNXLXNKXAFTXKXXYGXXEREAQWAXAQRTLHGLQXXEXXXXXFXXKXSYXXLSXIAEQAKRRAEXXRLREXXXLKXHVESVVKLKGLDIXTIXQXYTV

SEQ ID NO: 26 - protein, 106 aa, Artificial; identical to SEQ ID NO: 25
  Consensus sequence R1 domain
  VARIANT (4)..(4): Xaa can be replaced by  R, K
  VARIANT (7)..(7): Xaa can be replaced by  D, L, N, R
  VARIANT (9)..(9): Xaa can be replaced by  L, M
  VARIANT (11)..(11): Xaa can be replaced by  E, Q, D
  VARIANT (14)..(14): Xaa can be replaced by  T, I
  VARIANT (18)..(18): Xaa can be replaced by  T, S
  VARIANT (20)..(20): Xaa can be replaced by  K, E
  VARIANT (21)..(21): Xaa can be replaced by  D, N
  VARIANT (24)..(24): Xaa can be replaced by  K, R
  VARIANT (25)..(25): Xaa can be replaced by  E, G
  VARIANT (33)..(33): Xaa can be replaced by  T, A, L
  VARIANT (43)..(43): Xaa can be replaced by  P, A
  VARIANT (44)..(44): Xaa can be replaced by  P, A
  VARIANT (46)..(46): Xaa can be replaced by  T, V, A, P, K, S
  VARIANT (47)..(47): Xaa can be replaced by A, S, N
  VARIANT (48)..(48): Xaa can be replaced by  N, S, H
  VARIANT (49)..(49): :Xaa can be replaced by  N, T
  VARIANT (50)..(50): Xaa can be replaced by  I, V, M, L
  VARIANT (52)..(52): Xaa can be replaced by  N, S, H
  VARIANT (53)..(53): Xaa can be replaced by  E, D
  VARIANT (55)..(55): Xaa can be replaced by  S, N
  VARIANT (58)..(58): Xaa can be replaced by  R, S, H
  VARIANT (59)..(59): Xaa can be replaced by  E, D
  VARIANT (62)..(62): Xaa can be replaced by  E, Q
  VARIANT (73)..(73): Xaa can be replaced by  I, V, M
  VARIANT (74)..(74): Xaa can be replaced by  A, V
  VARIANT (79)..(79): Xaa can be replaced by  L, I, V
  VARIANT (80)..(80): Xaa can be replaced by  N, L, H
  VARIANT (81)..(81): Xaa can be replaced by  T, S
  VARIANT (84)..(84): Xaa can be replaced by  G, S
  VARIANT (98)..(98): Xaa can be replaced by  D, E
  VARIANT (101)..(101): Xaa can be replaced by  Q, N
  VARIANT (103)..(103): Xaa can be replaced by  N, H

SEQ ID NO: 27 - protein, 105 aa, Artificial
  Consensus sequence R1 domain
  VARIANT (4)..(4): Xaa can be replaced by  R, K
  VARIANT (7)..(7): Xaa can be replaced by  D, L, N, R
  VARIANT (9)..(9): Xaa can be replaced by  L, M
  VARIANT (11)..(11): Xaa can be replaced by  E, Q, D
  VARIANT (14)..(14): Xaa can be replaced by  T, I
  VARIANT (18)..(18): Xaa can be replaced by  T, S
  VARIANT (20)..(20): Xaa can be replaced by  K, E
  VARIANT (21)..(21): Xaa can be replaced by  D, N
  VARIANT (24)..(24): Xaa can be replaced by  K, R
  VARIANT (25)..(25): Xaa can be replaced by  E, G
  VARIANT (33)..(33): Xaa can be replaced by  T, A, L
  VARIANT (43)..(43): Xaa can be replaced by  P, A
  VARIANT (44)..(44): Xaa can be replaced by  P, A
  VARIANT (46)..(46): Xaa can be replaced by  T, V, A, P, K, S
  VARIANT (47)..(47): Xaa can be replaced by  N, S, H
  VARIANT (48)..(48): Xaa can be replaced by  N, T
  VARIANT (49)..(49): Xaa can be replaced by  I, V, M, L
  VARIANT (51)..(51): Xaa can be replaced by  N, S, H
  VARIANT (52)..(52): Xaa can be replaced by  E, D
  VARIANT (54)..(54): Xaa can be replaced by  S, N
  VARIANT (57)..(57): Xaa can be replaced by  R, S, H
  VARIANT (58)..(58): Xaa can be replaced by  E, D
  VARIANT (61)..(61): Xaa can be replaced by  E, Q
  VARIANT (72)..(72): Xaa can be replaced by  I, V, M
  VARIANT (73)..(73): Xaa can be replaced by  A, V
  VARIANT (78)..(78): Xaa can be replaced by  L, I, V
  VARIANT (79)..(79): Xaa can be replaced by  N, L, H
  VARIANT (80)..(80): Xaa can be replaced by  T, S
  VARIANT (83)..(83): Xaa can be replaced by  G, S
  VARIANT (97)..(97): Xaa can be replaced by  D, E
  VARIANT (100)..(100): Xaa can be replaced by  Q, N
  VARIANT (102)..(102): Xaa can be replaced by  N, H
LSGXAWXNXLXNKXAFTXKXXYGXXEREAQWAXAQRTLHGLQXXEXXXXFXXKXSYXXLSXIAEQAKRRAEXXRLREXXXLKXHVESVVKLKGLDIXTIXQXYTV

SEQ ID NO: 28 - protein, 107 aa, Artificial
  R1 domain mutated at position 31 W->L
  VARIANT (4)..(4): Xaa can be replaced by  R, K
  VARIANT (7)..(7): Xaa can be replaced by  D, L, N, R
  VARIANT (9)..(9): Xaa can be replaced by  L, M
  VARIANT (11)..(11): Xaa can be replaced by  E, Q, D
  VARIANT (14)..(14): Xaa can be replaced by  T, I
  VARIANT (18)..(18): Xaa can be replaced by  T, S
  VARIANT (20)..(20): Xaa can be replaced by  K, E
  VARIANT (21)..(21): Xaa can be replaced by  D, N
  VARIANT (24)..(24): Xaa can be replaced by  K, R
  VARIANT (25)..(25): Xaa can be replaced by  E, G
  VARIANT (33)..(33): Xaa can be replaced by  T, A, L
  VARIANT (43)..(43): Xaa can be replaced by  P, A
  VARIANT (44)..(44): Xaa can be replaced by  P, A
  VARIANT (46)..(46): Xaa can be replaced by  T, V, A, P, K, S
  VARIANT (47)..(47): Xaa can be replaced by A, S, N
  VARIANT (48)..(48): Xaa can be replaced by S, T, N
  VARIANT (49)..(49): Xaa can be replaced by  N, S, H
  VARIANT (50)..(50): Xaa can be replaced by  N, T
  VARIANT (51)..(51): Xaa can be replaced by  I, V, M, L
  VARIANT (53)..(53): Xaa can be replaced by  N, S, H
  VARIANT (54)..(54): Xaa can be replaced by  E, D
  VARIANT (56)..(56): Xaa can be replaced by  S, N
  VARIANT (59)..(59): Xaa can be replaced by  R, S, H
  VARIANT (60)..(60): Xaa can be replaced by  E, D
  VARIANT (63)..(63): Xaa can be replaced by  E, Q
  VARIANT (74)..(74): Xaa can be replaced by  I, V, M
  VARIANT (75)..(75): Xaa can be replaced by  A, V
  VARIANT (80)..(80): Xaa can be replaced by  L, I, V
  VARIANT (81)..(81): Xaa can be replaced by  N, L, H
  VARIANT (82)..(82): Xaa can be replaced by  T, S
  VARIANT (85)..(85): Xaa can be replaced by  G, S
  VARIANT (99)..(99): Xaa can be replaced by  D, E
  VARIANT (102)..(102): Xaa can be replaced by  Q, N
  VARIANT (104)..(104): Xaa can be replaced by  N, H
LSGXAWXNXLXNKXAFTXKXXYGXXEREAQLAXAQRTLHGLQXXEXXXXXXFXXKXSYXXLSXIAEQAKRRAEXXRLREXXXLKXHVESVVKLKGLDIXTIXQXYTV

SEQ ID NO: 29 - protein, 107 aa, Artificial
  R1 domain mutated at position 31 W->A
  VARIANT (4)..(4): Xaa can be replaced by  R, K
  VARIANT (7)..(7): Xaa can be replaced by  D, L, N, R
  VARIANT (9)..(9): Xaa can be replaced by  L, M
  VARIANT (11)..(11): Xaa can be replaced by  E, Q, D
  VARIANT (14)..(14): Xaa can be replaced by  T, I
  VARIANT (18)..(18): Xaa can be replaced by  T, S
  VARIANT (20)..(20): Xaa can be replaced by  K, E
  VARIANT (21)..(21): Xaa can be replaced by  D, N
  VARIANT (24)..(24): Xaa can be replaced by  K, R
  VARIANT (25)..(25): Xaa can be replaced by  E, G
  VARIANT (33)..(33): Xaa can be replaced by  T, A, L
  VARIANT (43)..(43): Xaa can be replaced by  P, A
  VARIANT (44)..(44): Xaa can be replaced by  P, A
  VARIANT (46)..(46): Xaa can be replaced by  T, V, A, P, K, S
  VARIANT (47)..(47): Xaa can be replaced by A, S, N
  VARIANT (48)..(48): Xaa can be replaced by S, T, N
  VARIANT (49)..(49): Xaa can be replaced by  N, S, H
  VARIANT (50)..(50): Xaa can be replaced by  N, T
  VARIANT (51)..(51): Xaa can be replaced by  I, V, M, L
  VARIANT (53)..(53): Xaa can be replaced by  N, S, H
  VARIANT (54)..(54): Xaa can be replaced by  E, D
  VARIANT (56)..(56): Xaa can be replaced by  S, N
  VARIANT (59)..(59): Xaa can be replaced by  R, S, H
  VARIANT (60)..(60): Xaa can be replaced by  E, D
  VARIANT (63)..(63): Xaa can be replaced by  E, Q
  VARIANT (74)..(74): Xaa can be replaced by  I, V, M
  VARIANT (75)..(75): Xaa can be replaced by  A, V
  VARIANT (80)..(80): Xaa can be replaced by  L, I, V
  VARIANT (81)..(81): Xaa can be replaced by  N, L, H
  VARIANT (82)..(82): Xaa can be replaced by  T, S
  VARIANT (85)..(85): Xaa can be replaced by  G, S
  VARIANT (99)..(99): Xaa can be replaced by  D, E
  VARIANT (102)..(102): Xaa can be replaced by  Q, N
  VARIANT (104)..(104): Xaa can be replaced by  N, H
LSGXAWXNXLXNKXAFTXKXXYGXXEREAQAAXAQRTLHGLQXXEXXXXXXFXXKXSYXXLSXIAEQAKRRAEXXRLREXXXLKXHVESVVKLKGLDIXTIXQXYTV

SEQ ID NO: 30 - protein, 931 aa, Arabidopsis thaliana
  misc_feature: AtAHA5_W857L mutant
MEEVFEELKCTKQGLTANEASHRLDVFGPNKLEEKKESKLLKFLGFMWNPLSWVMEVAALMAIALANGGGRPPDWQDFVGIVCLLLINSTISFIEENNAGNAAAALMAGLAPKTKVLRDNQWSEQEASILVPGDVISIKLGDIIPADARLLDGDPLKIDQSSLTGESIPVTKNPSDEVFSGSICKQGEIEAIVIATGVHTFFGKAAHLVDNTNQIGHFQKVLTSIGNFCICSIALGIIVELLVMYPIQRRRYRDGIDNLLVLLIGGIPIAMPSVLSVTMATGSHRLFQQGAITKRMTAIEEMAGMDVLCCDKTGTLTLNKLTVDKNLVEVFAKGVGKEHVFLLAARASRIENQDAIDAAIVGMLADPKEARAGVREVHFFPFNPVDKRTALTYVDSDGNWHRASKGAPEQILNLCNCKEDVRRKVHGVIDKFAERGLRSLAVARQEVLEKKKDAPGGPWQLVGLLPLFDPPRHDSAETIRRALNLGVNVKMITGDQLAIGKETGRRLGMGTNMYPSSALLGQVKDSSLGALPVDELIEKADGFAGVFPEHKYEIVHRLQQRNHICGMTGDGVNDAPALKKADIGIAVVDATDAARGASDIVLTEPGLSVIISAVLTSRAIFQRMKNYTIYAVSITIRIVFGFMFIALIWQFDFSPFMVLIIAILNDGTIMTISKDRMKPSPQPDSWKLRDIFSTGVVLGGYQALMTVVFFWVMKDSDFFSNYFGVRPLSQRPEQMMAALYLQVSIISQALIFVTRSRSWSYAECPGLLLLGAFVIAQLVATFIAVYANWSFARIEGAGWGWAGVIWLYSFLTYIPLDLLKFGIRYVLSGKAWLNLLENKTAFTTKKDYGKEEREAQLAAAQRTLHGLQPAEKNNIFNEKNSYSELSQIAEQAKRRAEVVRLREINTLKGHVESVVKLKGLDIDTIQQHYTV

SEQ ID NO: 31 - protein, 961 aa, Zea mays
  misc_feature: ZmAHA5_W885L mutant
MGPLQRRPTAMGGLEEIKNEAVDLENIPIEEVFEQLKCTREGLSSSEGQQRLEIFGPNRLEEKKESKILKFLGFMWNPLSWVMEMAAVMAIALANGGGKPPDWEDFVGIIVLLVINSTISFIEENNAGNAAAALMANLAPKTKVLRDGRWGEQEAAILVPGDIVSIKLGDIVPADARLLEGDPLKVDQSALTGESLPVTKGPGDEVFSGSTCKQGEIEAVVIATGVHTFFGKAAHLVDSTNQVGHFQQVLTAIGNFCICSIAVGIVVEIIVMFPIQHRRYRSGIENLLVLLIGGIPIAMPTVLSVTMAIGSHKLSQQGAITKRMTAIEEMAGMDVLCSDKTGTLTLNKLSVDKNLVEVFCKGVDKDHVLLLAARASRTENQDAIDAAMVGMLADPKEARAGIREIHFLPFNPVDKRTALTYIDADGHWHRVSKGAPEQILDLCHCKEDLRRKVHGIIDKYAERGLRSLAVARQEVPERNKESPGGPWQFVGLLPLFDPPRHDSAETIRKALVLGVNVKMITGDQLAIGKETGRRLGMGTNMYPSSALLGQNKDATLEALPVDELIEKADGFAGVFPEHKYEIVKRLQEKKHIVGMTGDGVNDAPALKKADIGIAVADATDAARSASDIVLTEPGLSVIISAVLTSRCIFQRMKNYTIYAVSITIRIVLGFMLIALIWQYDFSPFMVLIIAILNDGTIMTISKDRVKPSPLPDSWKLKEIFATGIVLGSYLALMTVIFFWAMHKTDFFSDKFGVRSIRDSEHEMMSALYLQVSIVSQALIFVTRSRSWSFVERPGLLLVTAFLLAQLVATFLAVYANWGFARIKGIGWGWAGVVWLYSIVFYFPLDLIKFFIRFVLSGRAWDNLLENKTAFTTKKDYGREEREAQLATAQRTLHGLQPPEAATSTLFHDKNSYRELSEIAEQAKRRAEIARLRELNTLKGHVESVVKLKGLDIDTIQQNYTV

SEQ ID NO: 32 - DNA, 40 bp, Artificial
  Amplification primer for the AtAHA5 gene
ggattctagaactagtatggaggaagtgttcgaggagctg

SEQ ID NO: 33 - DNA, 42 bp, Artificial
  Amplification primer for the AtAHA5 gene
cggtatcataagcttgttaaacggtgtaatgttgctgaatcg

SEQ ID NO: 34 - DNA, 27 bp, Artificial
  Primers for site directed mutagenesis of P50S
gggttcatgtggaactcattgtcgtgg

SEQ ID NO: 35 - DNA, 27 bp, Artificial
  Primers for site directed mutagenesis of P50S
ccacgacaatgagttccacatgaaccc

SEQ ID NO: 36 - DNA, 29 bp, Artificial
  Primers for site directed mutagenesis of W857L
ggaaagagaagctcaattggctgcagctc

SEQ ID NO: 37 - DNA, 29 bp, Artificial
  Primers for site directed mutagenesis of W857L
gagctgcagccaattgagcttctctttcc

SEQ ID NO: 38 - DNA, 48 bp, Artificial
  Amplification primer for the promoter pAtAHA5
ggggacaactttgtatagaaaagttgcaaccatcatgacaagcgtctg

SEQ ID NO: 39 - DNA, 52 bp, Artificial
  Amplification primer for the promoter pAtAHA5
ggggactgcttttttgtacaaacttggggtattcgtacctagacccatcatt

SEQ ID NO: 40 - DNA, 922 bp, Sorghum bicolor
  misc_feature: proSbMYB60
ctccgtcgctagcgttgtaatttttatcagcctctctccatctgattggatgagctgcttctcctagctagcacgttgtcaaccattggggacgccctttaggagtgaaagtgatgcagttactctactcccatccggtccaaatcccaacctaagggatatatgacgaagagttttcaatttcagtataatgtgtatagcaagtgatttgattttcctgcagattcttgagagagaagggccaaacctgcatatgtgccaggtgcgcactcacagtcacacacacggtcctcatcaatgcccaagaaatctggagagacacagacaaacgcaagcaattactccattcatgagcgccacagcagaaaaaggagtcctccagaaccggccgtgttcttggcttgcacacacacacacacacacgcgaaagcagcgcatgcaacaaagcaaagatcacacacggccggagcaagagagacgcccatattcatgtgatcacctggctgacttttgcattggaaagcaacagtgcgagatcaaaagcgaacgcagcacacagcacagcacagcacagggatcgagttgctctactccgtatatgaggtcatgcagtatataagcactcacatgcagctataccttagctagggcacctgtgcaaggggacaggtaggagataaagcaatgtctgctggctagaataaaaggaggccgatatcgtatcagcagagggttccaggggagaaggccgttctgcagggccgccgtaaaaggctgtgtaggaagcagccacagcttctcatatcttcttgttcttcgactacttgcctagctactatatctactagactagccctaggctgcttgctagctagtaggtgtatcgatcgtccgaggtaggaggagacagcaggaagcaggc

SEQ ID NO: 41 - DNA, 773 bp, Zea mays
  misc_feature: proZmMYB60
ggaagtgttttgattttcctgcagttctcgatcgagagaggccctcttgaatctgaaagaggtcgagaagggccagcctgcgtgtcccaggagcgtgcgctcacacacacggtcctcatcaatgcccaagaaatctggagagacacaaacaaacgcaaagcaattactcacttcatgagcgccacagcagaaaaggagtcctcaagcagtacgtcaaccggccgtgttctcgcacacgcaaaagcagcgcatgcaacaaagcaaagatcacacacccggagcgaagagacgcccattcatgtgatcacctggctgacttttgcattggaaagctacagtgcgagatcaaaagcgaacgcagcacagcacaggccgggggagtggcttatatgaggtcatgcagtatataagcactcacatgcagctagctaggtagagcacctgtgcatcaaggtaaagcagatggggcctgctctgctgcctgcctgcctgctggcatgcgtgtacgtcctagaataaaaggaggcccgtatcgtattagcagagggttccagggagaagagaagggagggcgaggccactggctgtgtaggcagcagccagccacacagacacagcttcgttcccatctcttctcgttcttcatcacctacttgcctactatatctactagccacgctagctagactagccttagaaaaggctagctcactagctgcttgctaggtgtgtaccgatcgtccgaggtaggagacacagcacgcagcaggggt

SEQ ID NO: 42 - DNA, 674 bp, Artificial
  pro35S
attgagacttttcaacaaagggtaatatccggaaacctcctcggattccattgcccagctatctgtcactttattgtgaagatagtggaaaaggaaggtggctcctacaaatgccatcattgcgataaaggaaaggccatcgttgaagatgcctctgccgacagtggtcccaaagatggacccccacccacgaggagcatcgtggaaaaagaagacgttccaaccacgtcttcaaagcaagtggattgatgtgataacatggtggagcacgacacacttgtctactccaaaaatatcaaagatacagtctcagaagaccaaagggcaattgagacttttcaacaaagggtaatatccggaaacctcctcggattccattgcccagctatctgtcactttattgtgaagatagtggaaaaggaaggtggctcctacaaatgccatcattgcgataaaggaaaggccatcgttgaagatgcctctgccgacagtggtcccaaagatggacccccacccacgaggagcatcgtggaaaaagaagacgttccaaccacgtcttcaaagcaagtggattgatgtgatatctccactgacgtaagggatgacgcacaatcccactatccttcgcaagacccttcctctatataaggaagttcatttcatttggagaggac

SEQ ID NO: 43 - DNA, 4023 bp, Artificial
  Cassette 35S-AtAHA5P50S
attgagacttttcaacaaagggtaatatccggaaacctcctcggattccattgcccagctatctgtcactttattgtgaagatagtggaaaaggaaggtggctcctacaaatgccatcattgcgataaaggaaaggccatcgttgaagatgcctctgccgacagtggtcccaaagatggacccccacccacgaggagcatcgtggaaaaagaagacgttccaaccacgtcttcaaagcaagtggattgatgtgataacatggtggagcacgacacacttgtctactccaaaaatatcaaagatacagtctcagaagaccaaagggcaattgagacttttcaacaaagggtaatatccggaaacctcctcggattccattgcccagctatctgtcactttattgtgaagatagtggaaaaggaaggtggctcctacaaatgccatcattgcgataaaggaaaggccatcgttgaagatgcctctgccgacagtggtcccaaagatggacccccacccacgaggagcatcgtggaaaaagaagacgttccaaccacgtcttcaaagcaagtggattgatgtgatatctccactgacgtaagggatgacgcacaatcccactatccttcgcaagacccttcctctatataaggaagttcatttcatttggagaggacctcgactctagaggatccccgggtaccgggccccccctcgaggcgcgccaaataatgattttattttgactgatagtgacctgttcgttgcaacaaattgatgagcaatgcttttttataatgccaactttgtacaaaaaagcaggctccatggaggaagtgttcgaggagctgaaatgtacaaaacaaggtcttacggcaaatgaagcttctcaccgtcttgacgtttttggtcctaacaagcttgaagagaagaaggaaagcaagttacttaagtttttagggttcatgtggaactcattgtcgtgggtgatggaggtggctgcactaatggcaatcgctttggccaacggaggaggacggccaccggattggcaagactttgtggggatagtgtgtttactattaatcaactcaaccattagtttcattgaggaaaataacgccggtaatgctgcagccgctctcatggccggtctagcccctaagacaaaggttctcagagataatcaatggagcgagcaagaagcatcgattctcgtccccggagatgtaatcagcatcaagctcggcgatatcattcccgccgatgcacgtttactcgacggcgatcctctcaaaatcgatcaatcatcactcaccggtgaatcaatccccgtcacaaaaaaccccagcgatgaagtcttctccggctcaatatgcaaacaaggcgaaatcgaagcaatcgtcatcgccactggagtccacacattcttcggcaaagcagctcatctcgtcgacaacacaaaccaaatcggccatttccagaaagttctcacttcgattggtaacttctgtatctgttcgattgctttaggaatcatcgttgagcttttagtaatgtatccgattcaacgccggagatatcgagacggaatcgataatttacttgttttgttgatcggagggattcctatagctatgcctagtgtgttatctgttacaatggcgactggttctcatagattgtttcaacaaggagctattactaagagaatgactgctattgaggaaatggctggtatggatgtattgtgttgtgataagactggtactcttacgcttaataagcttacggttgataagaacttagtcgaggttttcgctaaaggagttggtaaagaacatgttttccttttggctgcgagagcttcgaggattgagaatcaagatgcgattgatgctgctattgttggaatgcttgctgatcctaaagaggctagagctggtgttagagaggttcattttttcccttttaatccggttgataagagaactgctttgacttatgttgactctgatggaaactggcatagagctagtaaaggagctccagagcagatactgaacctctgtaattgcaaggaagatgttaggaggaaagttcatggagtgattgataagtttgctgagcgtggacttcgctctttggctgttgcaagacaggaagttctcgagaagaagaaagatgctcctggtggcccatggcaacttgtaggtcttttacctctttttgatcctccgaggcatgacagtgccgagacaatcaggagggctttaaacctcggtgttaatgttaagatgataaccggggaccagcttgcaattgggaaagagaccggtcgaaggcttggaatgggtacgaacatgtatccttcttctgcgctgctcggacaagtcaaagattcttccttgggtgcacttcctgtggatgaactgatagagaaggctgatgggtttgcaggagtctttccagaacataagtatgagattgttcataggctgcaacaaaggaatcacatatgtggcatgactggagatggtgtgaatgatgccccggctctcaagaaggcggatattggtatagctgttgttgatgctactgatgctgcgagaggcgcttctgatatcgttctcacagaacccggattgagtgttatcattagtgctgtactcaccagtagagccatattccaaagaatgaaaaattacactatttatgcggtttcaatcacgatacgaattgtgtttggcttcatgttcattgccctcatatggcagttcgatttttcgcctttcatggttctgatcatagcaatcttaaacgacggaacaatcatgacaatatcaaaagacagaatgaagccatctccacagccagatagctggaaactcagagatatattctcgaccggcgtcgtgcttggaggttaccaggccttgatgacagtcgttttcttctgggtgatgaaagacagtgattttttctcgaactattttggtgtgagaccactgagccaacgtcctgaacaaatgatggctgctctgtatctacaagttagcatcataagccaggctctcatcttcgtcaccagatcccgtagctggtcctacgccgaatgccctggccttctcttacttggtgcatttgtcatagctcagctggtggcgacatttatagcagtttatgcaaactggagttttgcccggatagaaggagccggttggggatgggctggagtgatctggctatacagtttcctaacgtacatccctcttgacttactcaagtttggaatccgctatgttttgagtggaaaagcttggttaaatcttcttgagaacaagactgccttcacgacgaagaaagactatgggaaagaggaaagagaagctcaatgggctgcagctcaaagaaccctccacggacttcaaccagcagagaaaaacaacatctttaacgaaaagaatagttacagtgaactctctcagattgctgaacaggctaaacgccgagctgaggttgtcaggctgagagagataaatacattaaaagggcatgtagagtcagtggtgaagcttaaaggacttgacattgacacgattcagcaacattacaccgtttaaaacccagctttcttgtacaaagttggcattataagaaagcattgcttatcaatttgttgcaacgaacaggtcactatcagtcaaaataaaatcattatttgttaattaactagttctagagcggccgcccaccgcggtggagctcgaatttccccgatcgttcaaacatttggcaataaagtttcttaagattgaatcctgttgccggtcttgcgatgattatcatataatttctgttgaattacgttaagcatgtaataattaacatgtaatgcatgacgttatttatgagatgggtttttatgattagagtcccgcaattatacatttaatacgcgatagaaaacaaaatatagcgcgcaaactaggataaattatcgcgcgcggtgtcatctatgttact

SEQ ID NO: 44 - DNA, 4023 bp, Artificial
  Cassette 35S-AtAHA5W857L
attgagacttttcaacaaagggtaatatccggaaacctcctcggattccattgcccagctatctgtcactttattgtgaagatagtggaaaaggaaggtggctcctacaaatgccatcattgcgataaaggaaaggccatcgttgaagatgcctctgccgacagtggtcccaaagatggacccccacccacgaggagcatcgtggaaaaagaagacgttccaaccacgtcttcaaagcaagtggattgatgtgataacatggtggagcacgacacacttgtctactccaaaaatatcaaagatacagtctcagaagaccaaagggcaattgagacttttcaacaaagggtaatatccggaaacctcctcggattccattgcccagctatctgtcactttattgtgaagatagtggaaaaggaaggtggctcctacaaatgccatcattgcgataaaggaaaggccatcgttgaagatgcctctgccgacagtggtcccaaagatggacccccacccacgaggagcatcgtggaaaaagaagacgttccaaccacgtcttcaaagcaagtggattgatgtgatatctccactgacgtaagggatgacgcacaatcccactatccttcgcaagacccttcctctatataaggaagttcatttcatttggagaggacctcgactctagaggatccccgggtaccgggccccccctcgaggcgcgccaaataatgattttattttgactgatagtgacctgttcgttgcaacaaattgatgagcaatgcttttttataatgccaactttgtacaaaaaagcaggctccatggaggaagtgttcgaggagctgaaatgtacaaaacaaggtcttacggcaaatgaagcttctcaccgtcttgacgtttttggtcctaacaagcttgaagagaagaaggaaagcaagttacttaagtttttagggttcatgtggaacccattgtcgtgggtgatggaggtggctgcactaatggcaatcgctttggccaacggaggaggacggccaccggattggcaagactttgtggggatagtgtgtttactattaatcaactcaaccattagtttcattgaggaaaataacgccggtaatgctgcagccgctctcatggccggtctagcccctaagacaaaggttctcagagataatcaatggagcgagcaagaagcatcgattctcgtccccggagatgtaatcagcatcaagctcggcgatatcattcccgccgatgcacgtttactcgacggcgatcctctcaaaatcgatcaatcatcactcaccggtgaatcaatccccgtcacaaaaaaccccagcgatgaagtcttctccggctcaatatgcaaacaaggcgaaatcgaagcaatcgtcatcgccactggagtccacacattcttcggcaaagcagctcatctcgtcgacaacacaaaccaaatcggccatttccagaaagttctcacttcgattggtaacttctgtatctgttcgattgctttaggaatcatcgttgagcttttagtaatgtatccgattcaacgccggagatatcgagacggaatcgataatttacttgttttgttgatcggagggattcctatagctatgcctagtgtgttatctgttacaatggcgactggttctcatagattgtttcaacaaggagctattactaagagaatgactgctattgaggaaatggctggtatggatgtattgtgttgtgataagactggtactcttacgcttaataagcttacggttgataagaacttagtcgaggttttcgctaaaggagttggtaaagaacatgttttccttttggctgcgagagcttcgaggattgagaatcaagatgcgattgatgctgctattgttggaatgcttgctgatcctaaagaggctagagctggtgttagagaggttcattttttcccttttaatccggttgataagagaactgctttgacttatgttgactctgatggaaactggcatagagctagtaaaggagctccagagcagatactgaacctctgtaattgcaaggaagatgttaggaggaaagttcatggagtgattgataagtttgctgagcgtggacttcgctctttggctgttgcaagacaggaagttctcgagaagaagaaagatgctcctggtggcccatggcaacttgtaggtcttttacctctttttgatcctccgaggcatgacagtgccgagacaatcaggagggctttaaacctcggtgttaatgttaagatgataaccggggaccagcttgcaattgggaaagagaccggtcgaaggcttggaatgggtacgaacatgtatccttcttctgcgctgctcggacaagtcaaagattcttccttgggtgcacttcctgtggatgaactgatagagaaggctgatgggtttgcaggagtctttccagaacataagtatgagattgttcataggctgcaacaaaggaatcacatatgtggcatgactggagatggtgtgaatgatgccccggctctcaagaaggcggatattggtatagctgttgttgatgctactgatgctgcgagaggcgcttctgatatcgttctcacagaacccggattgagtgttatcattagtgctgtactcaccagtagagccatattccaaagaatgaaaaattacactatttatgcggtttcaatcacgatacgaattgtgtttggcttcatgttcattgccctcatatggcagttcgatttttcgcctttcatggttctgatcatagcaatcttaaacgacggaacaatcatgacaatatcaaaagacagaatgaagccatctccacagccagatagctggaaactcagagatatattctcgaccggcgtcgtgcttggaggttaccaggccttgatgacagtcgttttcttctgggtgatgaaagacagtgattttttctcgaactattttggtgtgagaccactgagccaacgtcctgaacaaatgatggctgctctgtatctacaagttagcatcataagccaggctctcatcttcgtcaccagatcccgtagctggtcctacgccgaatgccctggccttctcttacttggtgcatttgtcatagctcagctggtggcgacatttatagcagtttatgcaaactggagttttgcccggatagaaggagccggttggggatgggctggagtgatctggctatacagtttcctaacgtacatccctcttgacttactcaagtttggaatccgctatgttttgagtggaaaagcttggttaaatcttcttgagaacaagactgccttcacgacgaagaaagactatgggaaagaggaaagagaagctcaattggctgcagctcaaagaaccctccacggacttcaaccagcagagaaaaacaacatctttaacgaaaagaatagttacagtgaactctctcagattgctgaacaggctaaacgccgagctgaggttgtcaggctgagagagataaatacattaaaagggcatgtagagtcagtggtgaagcttaaaggacttgacattgacacgattcagcaacattacaccgtttaaaacccagctttcttgtacaaagttggcattataagaaagcattgcttatcaatttgttgcaacgaacaggtcactatcagtcaaaataaaatcattatttgttaattaactagttctagagcggccgcccaccgcggtggagctcgaatttccccgatcgttcaaacatttggcaataaagtttcttaagattgaatcctgttgccggtcttgcgatgattatcatataatttctgttgaattacgttaagcatgtaataattaacatgtaatgcatgacgttatttatgagatgggtttttatgattagagtcccgcaattatacatttaatacgcgatagaaaacaaaatatagcgcgcaaactaggataaattatcgcgcgcggtgtcatctatgttact

SEQ ID NO: 45 - DNA, 4023 bp, Artificial
  Cassette 35S-AtAHA5 WT
attgagacttttcaacaaagggtaatatccggaaacctcctcggattccattgcccagctatctgtcactttattgtgaagatagtggaaaaggaaggtggctcctacaaatgccatcattgcgataaaggaaaggccatcgttgaagatgcctctgccgacagtggtcccaaagatggacccccacccacgaggagcatcgtggaaaaagaagacgttccaaccacgtcttcaaagcaagtggattgatgtgataacatggtggagcacgacacacttgtctactccaaaaatatcaaagatacagtctcagaagaccaaagggcaattgagacttttcaacaaagggtaatatccggaaacctcctcggattccattgcccagctatctgtcactttattgtgaagatagtggaaaaggaaggtggctcctacaaatgccatcattgcgataaaggaaaggccatcgttgaagatgcctctgccgacagtggtcccaaagatggacccccacccacgaggagcatcgtggaaaaagaagacgttccaaccacgtcttcaaagcaagtggattgatgtgatatctccactgacgtaagggatgacgcacaatcccactatccttcgcaagacccttcctctatataaggaagttcatttcatttggagaggacctcgactctagaggatccccgggtaccgggccccccctcgaggcgcgccaaataatgattttattttgactgatagtgacctgttcgttgcaacaaattgatgagcaatgcttttttataatgccaactttgtacaaaaaagcaggctccatggaggaagtgttcgaggagctgaaatgtacaaaacaaggtcttacggcaaatgaagcttctcaccgtcttgacgtttttggtcctaacaagcttgaagagaagaaggaaagcaagttacttaagtttttagggttcatgtggaacccattgtcgtgggtgatggaggtggctgcactaatggcaatcgctttggccaacggaggaggacggccaccggattggcaagactttgtggggatagtgtgtttactattaatcaactcaaccattagtttcattgaggaaaataacgccggtaatgctgcagccgctctcatggccggtctagcccctaagacaaaggttctcagagataatcaatggagcgagcaagaagcatcgattctcgtccccggagatgtaatcagcatcaagctcggcgatatcattcccgccgatgcacgtttactcgacggcgatcctctcaaaatcgatcaatcatcactcaccggtgaatcaatccccgtcacaaaaaaccccagcgatgaagtcttctccggctcaatatgcaaacaaggcgaaatcgaagcaatcgtcatcgccactggagtccacacattcttcggcaaagcagctcatctcgtcgacaacacaaaccaaatcggccatttccagaaagttctcacttcgattggtaacttctgtatctgttcgattgctttaggaatcatcgttgagcttttagtaatgtatccgattcaacgccggagatatcgagacggaatcgataatttacttgttttgttgatcggagggattcctatagctatgcctagtgtgttatctgttacaatggcgactggttctcatagattgtttcaacaaggagctattactaagagaatgactgctattgaggaaatggctggtatggatgtattgtgttgtgataagactggtactcttacgcttaataagcttacggttgataagaacttagtcgaggttttcgctaaaggagttggtaaagaacatgttttccttttggctgcgagagcttcgaggattgagaatcaagatgcgattgatgctgctattgttggaatgcttgctgatcctaaagaggctagagctggtgttagagaggttcattttttcccttttaatccggttgataagagaactgctttgacttatgttgactctgatggaaactggcatagagctagtaaaggagctccagagcagatactgaacctctgtaattgcaaggaagatgttaggaggaaagttcatggagtgattgataagtttgctgagcgtggacttcgctctttggctgttgcaagacaggaagttctcgagaagaagaaagatgctcctggtggcccatggcaacttgtaggtcttttacctctttttgatcctccgaggcatgacagtgccgagacaatcaggagggctttaaacctcggtgttaatgttaagatgataaccggggaccagcttgcaattgggaaagagaccggtcgaaggcttggaatgggtacgaacatgtatccttcttctgcgctgctcggacaagtcaaagattcttccttgggtgcacttcctgtggatgaactgatagagaaggctgatgggtttgcaggagtctttccagaacataagtatgagattgttcataggctgcaacaaaggaatcacatatgtggcatgactggagatggtgtgaatgatgccccggctctcaagaaggcggatattggtatagctgttgttgatgctactgatgctgcgagaggcgcttctgatatcgttctcacagaacccggattgagtgttatcattagtgctgtactcaccagtagagccatattccaaagaatgaaaaattacactatttatgcggtttcaatcacgatacgaattgtgtttggcttcatgttcattgccctcatatggcagttcgatttttcgcctttcatggttctgatcatagcaatcttaaacgacggaacaatcatgacaatatcaaaagacagaatgaagccatctccacagccagatagctggaaactcagagatatattctcgaccggcgtcgtgcttggaggttaccaggccttgatgacagtcgttttcttctgggtgatgaaagacagtgattttttctcgaactattttggtgtgagaccactgagccaacgtcctgaacaaatgatggctgctctgtatctacaagttagcatcataagccaggctctcatcttcgtcaccagatcccgtagctggtcctacgccgaatgccctggccttctcttacttggtgcatttgtcatagctcagctggtggcgacatttatagcagtttatgcaaactggagttttgcccggatagaaggagccggttggggatgggctggagtgatctggctatacagtttcctaacgtacatccctcttgacttactcaagtttggaatccgctatgttttgagtggaaaagcttggttaaatcttcttgagaacaagactgccttcacgacgaagaaagactatgggaaagaggaaagagaagctcaatgggctgcagctcaaagaaccctccacggacttcaaccagcagagaaaaacaacatctttaacgaaaagaatagttacagtgaactctctcagattgctgaacaggctaaacgccgagctgaggttgtcaggctgagagagataaatacattaaaagggcatgtagagtcagtggtgaagcttaaaggacttgacattgacacgattcagcaacattacaccgtttaaaacccagctttcttgtacaaagttggcattataagaaagcattgcttatcaatttgttgcaacgaacaggtcactatcagtcaaaataaaatcattatttgttaattaactagttctagagcggccgcccaccgcggtggagctcgaatttccccgatcgttcaaacatttggcaataaagtttcttaagattgaatcctgttgccggtcttgcgatgattatcatataatttctgttgaattacgttaagcatgtaataattaacatgtaatgcatgacgttatttatgagatgggtttttatgattagagtcccgcaattatacatttaatacgcgatagaaaacaaaatatagcgcgcaaactaggataaattatcgcgcgcggtgtcatctatgttact

SEQ ID NO: 46 - DNA, 2356 bp, Arabidopsis thaliana
  misc_feature: pAtAHA5
aaccatcatgacaagcgtctggatttttggaatctaggattttttgaacatatagtgtggtgattttttggggagaagagatcattgttgatgtatgttgcctgagttatggccgcgacgaaaaaatagactgaaatgtgtgaaaagatggtataaatatctttacctaggtttctaggttttgattactgggcatgtgaaatgggttttaataaatgggcttgggcttgtaaaattgtggaattaagctattgtaatcacgcatatgagttatctaattggataacttattagattgtaataatgagggaaaaaaaaagattattataatgagaggtccacatttaaaatgatgtgacactcttagcaaataaatataacatggcaaaatttagaagtgttgtcaaaaaacgataagcgtaaaatggaaattgtgactgaaccaccataagaagcgtctggatttttggagtccgagagatttagaaagtggagtgtggttgttttttttagagggggaatgttgttgtttatgccattagagtcatggtggcgtcgaagaacaataagtatatgtgggaatcagagatgtgtgtaagagaaacaaaaatttatttggttgggttttgaattttcaagaaaatgttaaattatttcatcgagtttctttttttttctctatgttaggaaatggtatggtcaaaatctattgatgatggtgatgcctaacattaacaaaaccaatagaagggagacaagagacataagacatcttcttgaaattcatcaacattacaaacttactaaaactcctcctcccaatcccaaatgaatatgtacttcttaaagccacgtgtctttctctttttcattaatatttatttatttttttaaaatgtgaaattatttctttggtttaatatctctggatcattcttctacaatgatcacaagtatttagatcatgtgtaaatagtcccatcatgaagttttaattaccaatcggtattgcacatcaccgattggtactgatccacctgcacttttgtcgatcttttgggacaacgaaaaagaaactaatttaatatattttgttatccgctcgaagatattaattataagctttaatttggaacttctttatatcaattatatatatatataacttctttgttaatagaaaatgggaacgatccaaaacttaagacatttgatctccacaaggccgtcgacgtacagagaagaagaatggccaaaaataagtaaataaaagagaagaaaccgaggggaagatgattttgcattgccacgacccacgagcatccatcggccatcgcctttttggattcacatggcaaagacaaacttcgatcttccttttttctcgtgaagttattatctctctaatttctagtctggtcgaacctatatttcatcatatatatcattatttaattcatatgctgatgcatgggacattatcatgttaagtcattacaaaaaaataaaaataaaaataacttacgttggactctcagtttaccttctcctatggatttcacttccttgtataagaatatacatcttactcaaatcatgatttatatgcaattttcttttgtgagattttttttacatataaaccagaaatgttgaaagaagaatatccaaacacaacaaaataatagaagaaatctcacgtagaacatggaaatggaaaaagaagtgaactcgtgaaccgatatatttaccaaaagtgcacacatagacaagtctttctcattaaagcccaatttcacactttcacattttcgtgacgtcttttgaagttttgaatacgaattaatgttcatgtacgctataaagacctaaaaggttgtcatatttctccactttcatcttctcttcacaactatcctaaaccttttttccttttcttcttcttcactctctttcttcccggcgtcactatggcggctgccgccgggtaaaggcagcgaactcgaccacatcaagaatgaatccgttgatctggtatatatatttacgtcttcttagttttctattatctatatgttttaaaaaatctttggccctactaattttaaattttctgttacataaaagatacatatatgtatagtacgtaactagtaactactttgatctaatcagttaatatatttgtcccatgcgatttactcatgtttccattagaaatgattagtcaaaattatataaatgatgggtctaggtacgaataccctaatatatttgtcccatgcgatttactcatgtttccattagaaatgattagtcaaaattatataaatgatgggtctaggtacgaataccc

SEQ ID NO: 47 - DNA, 6253 bp, Artificial
  Cassette pAtAHA5-AtAHA5W857L
aaccatcatgacaagcgtctggatttttggaatctaggattttttgaacatatagtgtggtgattttttggggagaagagatcattgttgatgtatgttgcctgagttatggccgcgacgaaaaaatagactgaaatgtgtgaaaagatggtataaatatctttacctaggtttctaggttttgattactgggcatgtgaaatgggttttaataaatgggcttgggcttgtaaaattgtggaattaagctattgtaatcacgcatatgagttatctaattggataacttattagattgtaataatgagggaaaaaaaaagattattataatgagaggtccacatttaaaatgatgtgacactcttagcaaataaatataacatggcaaaatttagaagtgttgtcaaaaaacgataagcgtaaaatggaaattgtgactgaaccaccataagaagcgtctggatttttggagtccgagagatttagaaagtggagtgtggttgttttttttagagggggaatgttgttgtttatgccattagagtcatggtggcgtcgaagaacaataagtatatgtgggaatcagagatgtgtgtaagagaaacaaaaatttatttggttgggttttgaattttcaagaaaatgttaaattatttcatcgagtttctttttttttctctatgttaggaaatggtatggtcaaaatctattgatgatggtgatgcctaacattaacaaaaccaatagaagggagacaagagacataagacatcttcttgaaattcatcaacattacaaacttactaaaactcctcctcccaatcccaaatgaatatgtacttcttaaagccacgtgtctttctctttttcattaatatttatttatttttttaaaatgtgaaattatttctttggtttaatatctctggatcattcttctacaatgatcacaagtatttagatcatgtgtaaatagtcccatcatgaagttttaattaccaatcggtattgcacatcaccgattggtactgatccacctgcacttttgtcgatcttttgggacaacgaaaaagaaactaatttaatatattttgttatccgctcgaagatattaattataagctttaatttggaacttctttatatcaattatatatatatataacttctttgttaatagaaaatgggaacgatccaaaacttaagacatttgatctccacaaggccgtcgacgtacagagaagaagaatggccaaaaataagtaaataaaagagaagaaaccgaggggaagatgattttgcattgccacgacccacgagcatccatcggccatcgcctttttggattcacatggcaaagacaaacttcgatcttccttttttctcgtgaagttattatctctctaatttctagtctggtcgaacctatatttcatcatatatatcattatttaattcatatgctgatgcatgggacattatcatgttaagtcattacaaaaaaataaaaataaaaataacttacgttggactctcagtttaccttctcctatggatttcacttccttgtataagaatatacatcttactcaaatcatgatttatatgcaattttcttttgtgagattttttttacatataaaccagaaatgttgaaagaagaatatccaaacacaacaaaataatagaagaaatctcacgtagaacatggaaatggaaaaagaagtgaactcgtgaaccgatatatttaccaaaagtgcacacatagacaagtctttctcattaaagcccaatttcacactttcacattttcgtgacgtcttttgaagttttgaatacgaattaatgttcatgtacgctataaagacctaaaaggttgtcatatttctccactttcatcttctcttcacaactatcctaaaccttttttccttttcttcttcttcactctctttcttcccggcgtcactatggcggctgccgccgggtaaaggcagcgaactcgaccacatcaagaatgaatccgttgatctggtatatatatttacgtcttcttagttttctattatctatatgttttaaaaaatctttggccctactaattttaaattttctgttacataaaagatacatatatgtatagtacgtaactagtaactactttgatctaatcagttaatatatttgtcccatgcgatttactcatgtttccattagaaatgattagtcaaaattatataaatgatgggtctaggtacgaataccctaatatatttgtcccatgcgatttactcatgtttccattagaaatgattagtcaaaattatataaatgatgggtctaggtacgaatacccatgcaagtttgtacaaaaaagcaggcttaatggtgagcaagggcgaggagctgttcaccggggtggtgcccatcctggtcgagctggacggcgacgtaaacggccacaagttcagcgtgtccggcgagggcgagggcgatgccacctacggcaagctgaccctgaagttcatctgcaccaccggcaagctgcccgtgccctggcccaccctcgtgaccaccctgacctacggcgtgcagtgcttcagccgctaccccgaccacatgaagcagcacgacttcttcaagtccgccatgcccgaaggctacgtccaggagcgcaccatcttcttcaaggacgacggcaactacaagacccgcgccgaggtgaagttcgagggcgacaccctggtgaaccgcatcgagctgaagggcatcgacttcaaggaggacggcaacatcctggggcacaagctggagtacaactacaacagccacaacgtctatatcatggccgacaagcagaagaacggcatcaaggtgaacttcaagatccgccacaacatcgaggacggcagcgtgcagctcgccgaccactaccagcagaacacccccatcggcgacggccccgtgctgctgcccgacaaccactacctgagcacccagtccgccctgagcaaagaccccaacgagaagcgcgatcacatggtcctgctggagttcgtgaccgccgccgggatcactctcggcatggacgagctgtacaagtacccagctttcttgtacaaagtggctatggaggaagtgttcgaggagctgaaatgtacaaaacaaggtcttacggcaaatgaagcttctcaccgtcttgacgtttttggtcctaacaagcttgaagagaagaaggaaagcaagttacttaagtttttagggttcatgtggaacccattgtcgtgggtgatggaggtggctgcactaatggcaatcgctttggccaacggaggaggacggccaccggattggcaagactttgtggggatagtgtgtttactattaatcaactcaaccattagtttcattgaggaaaataacgccggtaatgctgcagccgctctcatggccggtctagcccctaagacaaaggttctcagagataatcaatggagcgagcaagaagcatcgattctcgtccccggagatgtaatcagcatcaagctcggcgatatcattcccgccgatgcacgtttactcgacggcgatcctctcaaaatcgatcaatcatcactcaccggtgaatcaatccccgtcacaaaaaaccccagcgatgaagtcttctccggctcaatatgcaaacaaggcgaaatcgaagcaatcgtcatcgccactggagtccacacattcttcggcaaagcagctcatctcgtcgacaacacaaaccaaatcggccatttccagaaagttctcacttcgattggtaacttctgtatctgttcgattgctttaggaatcatcgttgagcttttagtaatgtatccgattcaacgccggagatatcgagacggaatcgataatttacttgttttgttgatcggagggattcctatagctatgcctagtgtgttatctgttacaatggcgactggttctcatagattgtttcaacaaggagctattactaagagaatgactgctattgaggaaatggctggtatggatgtattgtgttgtgataagactggtactcttacgcttaataagcttacggttgataagaacttagtcgaggttttcgctaaaggagttggtaaagaacatgttttccttttggctgcgagagcttcgaggattgagaatcaagatgcgattgatgctgctattgttggaatgcttgctgatcctaaagaggctagagctggtgttagagaggttcattttttcccttttaatccggttgataagagaactgctttgacttatgttgactctgatggaaactggcatagagctagtaaaggagctccagagcagatactgaacctctgtaattgcaaggaagatgttaggaggaaagttcatggagtgattgataagtttgctgagcgtggacttcgctctttggctgttgcaagacaggaagttctcgagaagaagaaagatgctcctggtggcccatggcaacttgtaggtcttttacctctttttgatcctccgaggcatgacagtgccgagacaatcaggagggctttaaacctcggtgttaatgttaagatgataaccggggaccagcttgcaattgggaaagagaccggtcgaaggcttggaatgggtacgaacatgtatccttcttctgcgctgctcggacaagtcaaagattcttccttgggtgcacttcctgtggatgaactgatagagaaggctgatgggtttgcaggagtctttccagaacataagtatgagattgttcataggctgcaacaaaggaatcacatatgtggcatgactggagatggtgtgaatgatgccccggctctcaagaaggcggatattggtatagctgttgttgatgctactgatgctgcgagaggcgcttctgatatcgttctcacagaacccggattgagtgttatcattagtgctgtactcaccagtagagccatattccaaagaatgaaaaattacactatttatgcggtttcaatcacgatacgaattgtgtttggcttcatgttcattgccctcatatggcagttcgatttttcgcctttcatggttctgatcatagcaatcttaaacgacggaacaatcatgacaatatcaaaagacagaatgaagccatctccacagccagatagctggaaactcagagatatattctcgaccggcgtcgtgcttggaggttaccaggccttgatgacagtcgttttcttctgggtgatgaaagacagtgattttttctcgaactattttggtgtgagaccactgagccaacgtcctgaacaaatgatggctgctctgtatctacaagttagcatcataagccaggctctcatcttcgtcaccagatcccgtagctggtcctacgccgaatgccctggccttctcttacttggtgcatttgtcatagctcagctggtggcgacatttatagcagtttatgcaaactggagttttgcccggatagaaggagccggttggggatgggctggagtgatctggctatacagtttcctaacgtacatccctcttgacttactcaagtttggaatccgctatgttttgagtggaaaagcttggttaaatcttcttgagaacaagactgccttcacgacgaagaaagactatgggaaagaggaaagagaagctcaattggctgcagctcaaagaaccctccacggacttcaaccagcagagaaaaacaacatctttaacgaaaagaatagttacagtgaactctctcagattgctgaacaggctaaacgccgagctgaggttgtcaggctgagagagataaatacattaaaagggcatgtagagtcagtggtgaagcttaaaggacttgacattgacacgattcagcaacattacaccgtttaacaactttattatacatagttgataattcactggccgtcgttttacaacgtcgtgactgggaaaacgatctaactgactagccgcggccatggcggccgggagcggccatgctagagtccgcaaaaatcaccagtctctctctacaaatctatctctctctatttttctccagaataatgtgtgagtagttcccagataagggaattagggttcttatagggtttcgctcatgtgttgagcatataagaaacccttagtatgtatttgtatttgtaaaatacttctatcaataaaatttctaattcctaaaaccaaaatccagtgacct

SEQ ID NO: 48 - DNA, 6253 bp, Artificial
  Cassette pAtAHA5-AtAHA5 WT
aaccatcatgacaagcgtctggatttttggaatctaggattttttgaacatatagtgtggtgattttttggggagaagagatcattgttgatgtatgttgcctgagttatggccgcgacgaaaaaatagactgaaatgtgtgaaaagatggtataaatatctttacctaggtttctaggttttgattactgggcatgtgaaatgggttttaataaatgggcttgggcttgtaaaattgtggaattaagctattgtaatcacgcatatgagttatctaattggataacttattagattgtaataatgagggaaaaaaaaagattattataatgagaggtccacatttaaaatgatgtgacactcttagcaaataaatataacatggcaaaatttagaagtgttgtcaaaaaacgataagcgtaaaatggaaattgtgactgaaccaccataagaagcgtctggatttttggagtccgagagatttagaaagtggagtgtggttgttttttttagagggggaatgttgttgtttatgccattagagtcatggtggcgtcgaagaacaataagtatatgtgggaatcagagatgtgtgtaagagaaacaaaaatttatttggttgggttttgaattttcaagaaaatgttaaattatttcatcgagtttctttttttttctctatgttaggaaatggtatggtcaaaatctattgatgatggtgatgcctaacattaacaaaaccaatagaagggagacaagagacataagacatcttcttgaaattcatcaacattacaaacttactaaaactcctcctcccaatcccaaatgaatatgtacttcttaaagccacgtgtctttctctttttcattaatatttatttatttttttaaaatgtgaaattatttctttggtttaatatctctggatcattcttctacaatgatcacaagtatttagatcatgtgtaaatagtcccatcatgaagttttaattaccaatcggtattgcacatcaccgattggtactgatccacctgcacttttgtcgatcttttgggacaacgaaaaagaaactaatttaatatattttgttatccgctcgaagatattaattataagctttaatttggaacttctttatatcaattatatatatatataacttctttgttaatagaaaatgggaacgatccaaaacttaagacatttgatctccacaaggccgtcgacgtacagagaagaagaatggccaaaaataagtaaataaaagagaagaaaccgaggggaagatgattttgcattgccacgacccacgagcatccatcggccatcgcctttttggattcacatggcaaagacaaacttcgatcttccttttttctcgtgaagttattatctctctaatttctagtctggtcgaacctatatttcatcatatatatcattatttaattcatatgctgatgcatgggacattatcatgttaagtcattacaaaaaaataaaaataaaaataacttacgttggactctcagtttaccttctcctatggatttcacttccttgtataagaatatacatcttactcaaatcatgatttatatgcaattttcttttgtgagattttttttacatataaaccagaaatgttgaaagaagaatatccaaacacaacaaaataatagaagaaatctcacgtagaacatggaaatggaaaaagaagtgaactcgtgaaccgatatatttaccaaaagtgcacacatagacaagtctttctcattaaagcccaatttcacactttcacattttcgtgacgtcttttgaagttttgaatacgaattaatgttcatgtacgctataaagacctaaaaggttgtcatatttctccactttcatcttctcttcacaactatcctaaaccttttttccttttcttcttcttcactctctttcttcccggcgtcactatggcggctgccgccgggtaaaggcagcgaactcgaccacatcaagaatgaatccgttgatctggtatatatatttacgtcttcttagttttctattatctatatgttttaaaaaatctttggccctactaattttaaattttctgttacataaaagatacatatatgtatagtacgtaactagtaactactttgatctaatcagttaatatatttgtcccatgcgatttactcatgtttccattagaaatgattagtcaaaattatataaatgatgggtctaggtacgaataccctaatatatttgtcccatgcgatttactcatgtttccattagaaatgattagtcaaaattatataaatgatgggtctaggtacgaatacccatgcaagtttgtacaaaaaagcaggcttaatggtgagcaagggcgaggagctgttcaccggggtggtgcccatcctggtcgagctggacggcgacgtaaacggccacaagttcagcgtgtccggcgagggcgagggcgatgccacctacggcaagctgaccctgaagttcatctgcaccaccggcaagctgcccgtgccctggcccaccctcgtgaccaccctgacctacggcgtgcagtgcttcagccgctaccccgaccacatgaagcagcacgacttcttcaagtccgccatgcccgaaggctacgtccaggagcgcaccatcttcttcaaggacgacggcaactacaagacccgcgccgaggtgaagttcgagggcgacaccctggtgaaccgcatcgagctgaagggcatcgacttcaaggaggacggcaacatcctggggcacaagctggagtacaactacaacagccacaacgtctatatcatggccgacaagcagaagaacggcatcaaggtgaacttcaagatccgccacaacatcgaggacggcagcgtgcagctcgccgaccactaccagcagaacacccccatcggcgacggccccgtgctgctgcccgacaaccactacctgagcacccagtccgccctgagcaaagaccccaacgagaagcgcgatcacatggtcctgctggagttcgtgaccgccgccgggatcactctcggcatggacgagctgtacaagtacccagctttcttgtacaaagtggctatggaggaagtgttcgaggagctgaaatgtacaaaacaaggtcttacggcaaatgaagcttctcaccgtcttgacgtttttggtcctaacaagcttgaagagaagaaggaaagcaagttacttaagtttttagggttcatgtggaacccattgtcgtgggtgatggaggtggctgcactaatggcaatcgctttggccaacggaggaggacggccaccggattggcaagactttgtggggatagtgtgtttactattaatcaactcaaccattagtttcattgaggaaaataacgccggtaatgctgcagccgctctcatggccggtctagcccctaagacaaaggttctcagagataatcaatggagcgagcaagaagcatcgattctcgtccccggagatgtaatcagcatcaagctcggcgatatcattcccgccgatgcacgtttactcgacggcgatcctctcaaaatcgatcaatcatcactcaccggtgaatcaatccccgtcacaaaaaaccccagcgatgaagtcttctccggctcaatatgcaaacaaggcgaaatcgaagcaatcgtcatcgccactggagtccacacattcttcggcaaagcagctcatctcgtcgacaacacaaaccaaatcggccatttccagaaagttctcacttcgattggtaacttctgtatctgttcgattgctttaggaatcatcgttgagcttttagtaatgtatccgattcaacgccggagatatcgagacggaatcgataatttacttgttttgttgatcggagggattcctatagctatgcctagtgtgttatctgttacaatggcgactggttctcatagattgtttcaacaaggagctattactaagagaatgactgctattgaggaaatggctggtatggatgtattgtgttgtgataagactggtactcttacgcttaataagcttacggttgataagaacttagtcgaggttttcgctaaaggagttggtaaagaacatgttttccttttggctgcgagagcttcgaggattgagaatcaagatgcgattgatgctgctattgttggaatgcttgctgatcctaaagaggctagagctggtgttagagaggttcattttttcccttttaatccggttgataagagaactgctttgacttatgttgactctgatggaaactggcatagagctagtaaaggagctccagagcagatactgaacctctgtaattgcaaggaagatgttaggaggaaagttcatggagtgattgataagtttgctgagcgtggacttcgctctttggctgttgcaagacaggaagttctcgagaagaagaaagatgctcctggtggcccatggcaacttgtaggtcttttacctctttttgatcctccgaggcatgacagtgccgagacaatcaggagggctttaaacctcggtgttaatgttaagatgataaccggggaccagcttgcaattgggaaagagaccggtcgaaggcttggaatgggtacgaacatgtatccttcttctgcgctgctcggacaagtcaaagattcttccttgggtgcacttcctgtggatgaactgatagagaaggctgatgggtttgcaggagtctttccagaacataagtatgagattgttcataggctgcaacaaaggaatcacatatgtggcatgactggagatggtgtgaatgatgccccggctctcaagaaggcggatattggtatagctgttgttgatgctactgatgctgcgagaggcgcttctgatatcgttctcacagaacccggattgagtgttatcattagtgctgtactcaccagtagagccatattccaaagaatgaaaaattacactatttatgcggtttcaatcacgatacgaattgtgtttggcttcatgttcattgccctcatatggcagttcgatttttcgcctttcatggttctgatcatagcaatcttaaacgacggaacaatcatgacaatatcaaaagacagaatgaagccatctccacagccagatagctggaaactcagagatatattctcgaccggcgtcgtgcttggaggttaccaggccttgatgacagtcgttttcttctgggtgatgaaagacagtgattttttctcgaactattttggtgtgagaccactgagccaacgtcctgaacaaatgatggctgctctgtatctacaagttagcatcataagccaggctctcatcttcgtcaccagatcccgtagctggtcctacgccgaatgccctggccttctcttacttggtgcatttgtcatagctcagctggtggcgacatttatagcagtttatgcaaactggagttttgcccggatagaaggagccggttggggatgggctggagtgatctggctatacagtttcctaacgtacatccctcttgacttactcaagtttggaatccgctatgttttgagtggaaaagcttggttaaatcttcttgagaacaagactgccttcacgacgaagaaagactatgggaaagaggaaagagaagctcaatgggctgcagctcaaagaaccctccacggacttcaaccagcagagaaaaacaacatctttaacgaaaagaatagttacagtgaactctctcagattgctgaacaggctaaacgccgagctgaggttgtcaggctgagagagataaatacattaaaagggcatgtagagtcagtggtgaagcttaaaggacttgacattgacacgattcagcaacattacaccgtttaacaactttattatacatagttgataattcactggccgtcgttttacaacgtcgtgactgggaaaacgatctaactgactagccgcggccatggcggccgggagcggccatgctagagtccgcaaaaatcaccagtctctctctacaaatctatctctctctatttttctccagaataatgtgtgagtagttcccagataagggaattagggttcttatagggtttcgctcatgtgttgagcatataagaaacccttagtatgtatttgtatttgtaaaatacttctatcaataaaatttctaattcctaaaaccaaaatccagtgacct

SEQ ID NO: 49 - DNA, 2886 bp, Zea mays
  misc_feature: ZmAHA5W885L version 1
atggggccactgcagcggcggcctacggctatgggggggctggaggagattaagaacgaggcggttgacctggagaacatcccgattgaggaggtgttcgagcagctgaagtgcacccgcgagggcctctccagctcggaggggcagcagcgcctggagatcttcggccccaaccgcctggaggagaagaaggagtccaagatcctcaagttcctgggcttcatgtggaacccactgagctgggttatggagatggctgccgtgatggctatcgcgctcgctaatggcgggggcaagccaccagactgggaggatttcgtcggcatcattgtgctcctggtcatcaactcgacgatttctttcatcgaggagaacaatgctggcaacgctgccgcggctctgatggctaatctcgctcctaagacaaaggtgctgagggatggccgctggggggagcaggaggccgcgatcctggtgccgggcgacattgtcagcatcaagctcggggacatcgttccagctgatgctaggctcctggagggggacccactcaaggtggatcagagcgctctgacgggcgagtcgctccctgtcacaaaggggccaggcgacgaggttttctccggcagcacgtgcaagcagggggagattgaggccgtggtcatcgcgactggcgtccacaccttcttcgggaaggctgcccatctggtcgactcgactaaccaggttggccacttccagcaggtgctcaccgcgatcgggaatttctgcatttgctctatcgctgtgggcattgttgtggagatcattgtcatgttcccaatccagcataggcgctaccgctccggcattgagaacctcctggtgctcctgatcgggggcatccccattgcgatgccaacggttctgagcgtgacaatggccatcggcagccacaagctctcgcagcagggggccattacgaagaggatgacagccatcgaggagatggcggggatggacgtcctgtgctctgataagacaggcactctcaccctgaacaagctgtcagtggacaagaatctcgttgaggtgttctgcaagggcgttgacaaggatcacgtgctcctgctcgcggctcgggcctcccgcaccgagaaccaggacgcgatcgatgctgcgatggtggggatgctcgccgatccaaaggaggctagggccggcattcgggagatccatttcctgcccttcaatccagtcgacaagaggactgctctcacctacatcgacgccgatggccactggcatcgggtgagcaagggggccccagagcagatcctcgacctgtgccactgcaaggaggatctgcggcgcaaggtgcatggcatcattgacaagtacgcggagagggggctcaggtcgctggcggtcgctcggcaggaggttcccgagcgcaacaaggagtctcctgggggcccgtggcagttcgtcggcctgctcccactcttcgacccacctcggcacgattccgcggagactatccgcaaggctctcgtgctgggcgtcaatgttaagatgattaccggggatcagctggccatcggcaaggagacggggaggaggctcgggatgggcacaaacatgtacccgtcttcagcgctgctcggccagaataaggacgctaccctggaggccctcccggtggacgagctgatcgagaaggcggatggcttcgctggggtcttcccggagcacaagtacgagattgttaagaggctgcaggagaagaagcatatcgtgggcatgacgggggacggcgtcaacgatgctcctgctctcaagaaggcggatatcggcattgctgtcgctgacgctacggatgctgctcggtcggcctctgacatcgttctgacagagccgggcctctctgtgatcatttcagcggtcctgacctcacgctgcattttccagaggatgaagaactacactatctacgcggtttccatcaccattcgcatcgtgctcggcttcatgctcattgccctgatctggcagtacgacttctctccgttcatggtcctgatcattgccatcctcaatgacggcacgattatgacaatctcaaaggatagggtgaagccatcgcctctgccggactcttggaagctcaaggagattttcgccacaggcatcgtgctggggtcctacctcgctctgatgactgtcatcttcttctgggccatgcacaagaccgacttcttcagcgataagttcggcgtccgctccatcagggacagcgagcatgagatgatgtcggcgctctacctgcaggtctcaattgtttcccaggccctcatcttcgtgacccggtcacgctcctggagcttcgttgagaggccaggcctgctcctggtgacggccttcctcctggcgcagctggtcgctacattcctcgccgtttacgcgaactggggcttcgcgcgcattaaggggatcggctgggggtgggctggcgtcgtttggctgtactccatcgtcttctacttcccgctcgacctgattaagttcttcatcaggttcgtgctcagcggccgggcgtgggataacctcctggagaataagacggccttcaccacgaagaaggactacggcagggaggagcgcgaggctcagctcgctactgctcagcgcaccctccacggcctgcagccaccagaggctgctacgtcgacactgttccatgacaagaactcatacagggagctctccgagattgctgagcaggccaagcgcagggcggagatcgctaggctcagggagctgaacaccctcaaggggcacgtcgagtccgtggtcaagctgaagggcctcgacattgatactatccagcagaattacaccgtgtag

SEQ ID NO: 50 - DNA, 2886 bp, Zea mays
  misc_feature: ZmAHA5W885L version 2
atgggcccactgcagaggcgcccaacagcgatggggggcctggaggagatcaagaacgaggccgtcgatctggagaacatccctattgaggaggtgttcgagcagctgaagtgcacccgggagggcctcagctcctcggagggccagcagcgcctggagatcttcggcccaaaccggctggaggagaagaaggagagcaagatcctcaagttcctggggttcatgtggaacccgctgtcctgggtcatggagatggctgccgtgatggcgattgctctggctaatggcgggggcaagccaccggactgggaggatttcgtggggattatcgtcctgctcgtcatcaacagcactatctccttcattgaggagaacaacgctggcaacgccgctgctgcgctgatggcgaacctcgctccaaagactaaggtcctccgcgacggccgctggggggagcaggaggctgcgattctcgtgcccggggacatcgttagcattaagctcggggatatcgtccctgctgatgcccggctgctggagggggaccccctgaaggtcgaccagagcgctctcaccggcgagtcgctcccagtcactaagggccctggggacgaggtgttcagcggctctacgtgcaagcagggcgagatcgaggcggtcgtgatcgctaccggcgtgcacaccttcttcgggaaggccgcccatctcgtggattcgacaaaccaggtcgggcacttccagcaggtgctgacagccatcgggaacttctgcatctgctcgattgccgttgggatcgtggttgagattattgtgatgttcccgattcagcaccggcgctaccgctccgggatcgagaacctcctggtcctcctcattggggggattccgatcgctatgccgaccgtcctgagcgtcactatggctatcgggtctcacaagctctcacagcagggggcgattaccaagcggatgacagcgattgaggagatggcggggatggacgtgctgtgctcagacaagaccggcactctgacgctcaacaagctctccgtggacaagaacctcgtcgaggtgttctgcaagggggtggacaaggatcatgtcctgctgctggcggccagggcctcccggacagagaaccaggacgccattgacgccgctatggtggggatgctggccgaccctaaggaggcgagggccggcatccgcgagattcacttcctgccattcaatcccgttgacaagcgcactgcgctgacgtacattgatgcggacgggcactggcacagggtgtccaagggggctccagagcagatcctcgatctgtgccactgcaaggaggatctgcggcgcaaggtgcatgggatcattgacaagtacgcggagagggggctccggagcctggcggtggccaggcaggaggtgccggagcgcaacaaggagtcgccggggggcccttggcagttcgtcgggctgctccctctgttcgatcccccgaggcacgacagcgcggagactatccgcaaggccctcgttctgggggtgaatgtcaagatgattaccggggaccagctggccattgggaaggagacaggccggcgcctcgggatgggcacgaacatgtacccgtcatccgccctgctggggcagaataaggacgccactctggaggccctgccggtcgatgagctcatcgagaaggctgacgggttcgcgggcgtcttccccgagcataagtacgagatcgtgaagcggctgcaggagaagaagcatattgtggggatgactggcgacggggtgaatgatgctcccgccctgaagaaggctgacatcggcattgccgtcgcggacgccacagatgctgcccgctcggcgtccgatatcgttctcacggagcctgggctgagcgttattatctcggcggttctgacaagcaggtgcatcttccagcgcatgaagaactacaccatctacgctgtgtcgatcactatcaggatcgtgctgggcttcatgctgattgcgctcatctggcagtacgacttctcccctttcatggtcctgatcattgctatcctcaacgacggcacaatcatgactatctcgaaggaccgcgtgaagccgagcccactccccgactcttggaagctcaaggagattttcgccactgggatcgttctcgggtcttacctcgctctgatgaccgtgattttcttctgggctatgcacaagaccgacttcttcagcgacaagttcggggttcgctcgattcgcgactcggagcacgagatgatgtctgcgctgtacctccaggtttcaattgtttcacaggcgctcattttcgtgactaggtcacggtcttggtccttcgtcgagaggcctggcctgctcctggtcactgctttcctgctcgcccagctggtggccactttcctcgctgtttacgctaattgggggttcgctaggatcaaggggatcggctgggggtgggcgggcgtggtctggctctactccatcgttttctacttcccactcgacctcatcaagttcttcattcggttcgtgctgtcagggagggcgtgggacaacctcctggagaacaagaccgcgttcaccactaagaaggactacggccgcgaggagagggaggcgcagctggctacagcgcagcgcaccctccacgggctccagcccccagaggctgcgacatctacactcttccacgacaagaattcttaccgcgagctgtcagagattgccgagcaggctaagcgcagggcggagattgctaggctgagggagctcaacacactgaagggccacgtggagtcagtggtcaagctgaagggcctggacatcgatacaattcagcagaactacaccgtttag

SEQ ID NO: 51 - DNA, 504 bp, Cassava vein mosaic virus
  misc_feature: proCsVMV
aaggtaattatccaagatgtagcatcaagaatccaatgtttacgggaaaaactatggaagtattatgtgagctcagcaagaagcagatcaatatgcggcacatatgcaacctatgttcaaaaatgaagaatgtacagatacaagatcctatactgccagaatacgaagaagaatacgtagaaattgaaaaagaagaaccaggcgaagaaaagaatcttgaagacgtaagcactgacgacaacaatgaaaagaagaagataaggtcggtgattgtgaaagagacatagaggacacatgtaaggtggaaaatgtaagggcggaaagtaaccttatcacaaaggaatcttatcccccactacttatccttttatatttttccgtgtcatttttgcccttgagttttcctatataaggaaccaagttcggcatttgtgaaaacaagaaaaaatttggtgtaagctattttctttgaagtactgaggatacaacttcagagaaatttgt

SEQ ID NO: 52 - DNA, 557 bp, Artificial
  Rice actin intron
accaccaccaccaccaccacctccacctcctcccccctcgctgccggacgacgagctcctcccccctccccctccgccgccgccgcgccggtaaccaccccgcccctctcctctttctttctccgttttttttttccgtctcggtctcgatctttggccttggtagtttgggtgggcgagaggcggcttcgtgcgcgcccagatcggtgcgcgggaggggcgggatctcgcggctggggctctcgccggcgtggatccggcccggatctcgcggggaatggggctctcggatgtagatctgcgatccgccgttgttgggggagatgatggggggtttaaaatttccgccatgctaaacaagatcaggaagaggggaaaagggcactatggtttatatttttatatatttctgctgcttcgtcaggcttagatgtgctagatctttctttcttctttttgtgggtagaatttgaatccctcagcattgttcatcggtagtttttcttttcatgatttgtgacaaatgcagcctcgtgcggagcttttttgtaggtaga

SEQ ID NO: 53 - DNA, 509 bp, Arabidopsis thaliana
  misc_feature: terSac66
ctaaatgctcttaactgagctaattatgtaatgcacatacacatatttacatagatatgcatatttatatatagcatgtatattgtactacatgcattgcttcttaatacatgtagtaaagatatatgcaaaaatagtcgaaagatttgtttacatataaaatcaccaatatttattgttattgtattttcatgaataaagtaataagattatttgtctaatattttgatttactagtactagaaatgaaaaggaatatgcacaatttcagcattatagtttggtaggcaaaatggagtgagaatagagtttcatagtatatactaaggttcttaattgtgcaaatagttgatacaagtcacatgggccaagtttgtaaatcttaaatcgaaatatgccttcttctttttttgcatgaaaatgctagtaatttataagtgtgtttttcaataagagatgctaaataccaaaattaacctagttttcagtgagcgcttgcattattgtgg

SEQ ID NO: 54 - DNA, 968 bp, Zea mays
  misc_feature: proZmrbcS_Mut_al
tccctttaatctggcgctagatctgcatccgcggcttgcaaagataaatggcacatttagtgtgttattttgcaatacctttcatagtagatatccttaaatgcagttttaggcatgtttgggtaattaaataacatttttaggaggagttttagatttacctttctttcgtgatgactgatgacagacgtggggaattcaaatgcaactctagcgaaagttcatatatttttcataaatagctgaggctggggtaattattttttttgtagaaaaatagaataggtggaatggttggggaaggcgtaggcgctcgtggacgacgcccgataaaagacaagaggcggaattgccatgaattcgaggtagctaagtaaggcgcatatatatgccaaaaaattctactgtcactttccaatttcaatgcgctgccaaacaagccatcctggaaactgacttgaattcagcccaattctgtagatccaaacagggccggcgtcagtgcctcaggtgagagagcagcagacgattcaaagagccaaaactgcaagcagacgcagccgaagccgaagccgaagcccaagcccaaaactgttttgtctttgcccagaaccgcgacgagcctaaactgcgcttcctcctatctacaagtccctggcacatcacgcatagtccaacctaggcgcgcaggcgataaggcgcgccacggggacgcgacatgtggtggcggacgcgatcaggatagggccaggctggccgggcgcggccacgggagaacggtggccactcgtcccacatccgcttcgtcctgtcctgtactgcgtcctgcccccaacgagagccggagccggccatcccgtcgcacactctccccctctatatatgccgtcggtgtgggggagcctactacaggacgacccaagcaagcaagcaagcagcgagtacatacatactaggcagccaggcag

SEQ ID NO: 55 - DNA, 537 bp, Zea mays
  misc_feature: terZmRbcs
tagaccgcgcccgccggccgccccccgccggctagctagctagctagctagctcctgcgtgagctagtagctagtgccatgcgtcgtctctgtcgttcggttttgcttcgggtcaccgtaccctttgcttgcttggtttcttctttccttttttccttttttttttcttcttttccccggccatggttcctttgctttcagcagttctctgctggatgtgatgtatccattgttgcaagcatggccttgcattggctacctctatacctgctacaaactactgcaacgcctatatatacttggggtgaggaacatgtgaatgcaagctccggctatcatatacatgtaatatggatacaaactatatatataaatccgccgaggcgccgactaatactatacgacgacaccgtgttaagttaatatataactggtgctttttatttatatatctgtctcatcatatatatatgctaattaatggatgtgtgtcctcttcacttcaattccttctttcctttcctatgctttgagatc

SEQ ID NO: 56 - DNA, 444 bp, Zea mays
  misc_feature: proZmRAB17_del
aaatgttatgcagttcgctctggacttttctgctgcgcctacacttgggtgtactgggcctaaattcagcctgaccgaccgcctgcattgaataatggatgagcaccggtaaaatccgcgtacccaactttcgagaagaaccgagacgtggcgggccgggccaccgacgcacggcaccagcgactgcacacgtcccgccggcgtacgtgtacgtgctgttccctcactggccgcccaatccactcatgcatgcccacgtacacccctgccgtggcgcgcccagatcctaatcctttcgccgttctgcacttctgctgcctataaatggcggcatcgaccgtcacctgcttcaccaccggcgagccacatcgagaacacgatcgagcacacaagcacgaagactcgtttaggagaaaccacaaaccaccaagccgtgcaagcatc

SEQ ID NO: 57 - DNA, 500 bp, Zea mays
  misc_feature: terZmRab17
gcggcgcctatacgtggctgtgctgtgctgtctggcgcgtcaaagccgtactcttcagcgttccatagataataagataaacccatgaataagtgtccctaccctttgatcatgtgacagggacagggacagtttcctgtacttgtggggtgaatttgtacgtgtgatacggtaacttggtccgtgtactgtttatgctgctacgtttccttcctaaaagtacgtatatatatacagcacttgcgagtggctttacttgtgtgcactgcctaaaagtgtcgatattacctccagcggtaaataaatgacccttgtaagaaacttacacagcatgtcttactaattaacagccgttattatgttcggcgcagtactcacactggaacttacgaacaagaattgctctatcaatcaccatctactttagatatatcttctgaaacttttttcaaatccaaaagttcagtatcttcctacaaattagtgaattaggaatccaa

SEQ ID NO: 58 - DNA, 4416 bp, Artificial
  Cassette_T02781_CsVMV ZmAHA5_W885L
aaggtaattatccaagatgtagcatcaagaatccaatgtttacgggaaaaactatggaagtattatgtgagctcagcaagaagcagatcaatatgcggcacatatgcaacctatgttcaaaaatgaagaatgtacagatacaagatcctatactgccagaatacgaagaagaatacgtagaaattgaaaaagaagaaccaggcgaagaaaagaatcttgaagacgtaagcactgacgacaacaatgaaaagaagaagataaggtcggtgattgtgaaagagacatagaggacacatgtaaggtggaaaatgtaagggcggaaagtaaccttatcacaaaggaatcttatcccccactacttatccttttatatttttccgtgtcatttttgcccttgagttttcctatataaggaaccaagttcggcatttgtgaaaacaagaaaaaatttggtgtaagctattttctttgaagtactgaggatacaacttcagagaaatttgtccctcccccctccccctccgccgccgccgcgccggtaaccaccccgcccctctcctctttctttctccgttttttttttccgtctcggtctcgatctttggccttggtagtttgggtgggcgagaggcggcttcgtgcgcgcccagatcggtgcgcgggaggggcgggatctcgcggctggggctctcgccggcgtggatccggcccggatctcgcggggaatggggctctcggatgtagatctgcgatccgccgttgttgggggagatgatggggggtttaaaatttccgccatgctaaacaagatcaggaagaggggaaaagggcactatggtttatatttttatatatttctgctgcttcgtcaggcttagatgtgctagatctttctttcttctttttgtgggtagaatttgaatccctcagcattgttcatcggtagtttttcttttcatgatttgtgacaaatgcagcctcgtgcggagcttttttgtaggtagacgatatctccaccatggggccactgcagcggcggcctacggctatgggggggctggaggagattaagaacgaggcggttgacctggagaacatcccgattgaggaggtgttcgagcagctgaagtgcacccgcgagggcctctccagctcggaggggcagcagcgcctggagatcttcggccccaaccgcctggaggagaagaaggagtccaagatcctcaagttcctgggcttcatgtggaacccactgagctgggttatggagatggctgccgtgatggctatcgcgctcgctaatggcgggggcaagccaccagactgggaggatttcgtcggcatcattgtgctcctggtcatcaactcgacgatttctttcatcgaggagaacaatgctggcaacgctgccgcggctctgatggctaatctcgctcctaagacaaaggtgctgagggatggccgctggggggagcaggaggccgcgatcctggtgccgggcgacattgtcagcatcaagctcggggacatcgttccagctgatgctaggctcctggagggggacccactcaaggtggatcagagcgctctgacgggcgagtcgctccctgtcacaaaggggccaggcgacgaggttttctccggcagcacgtgcaagcagggggagattgaggccgtggtcatcgcgactggcgtccacaccttcttcgggaaggctgcccatctggtcgactcgactaaccaggttggccacttccagcaggtgctcaccgcgatcgggaatttctgcatttgctctatcgctgtgggcattgttgtggagatcattgtcatgttcccaatccagcataggcgctaccgctccggcattgagaacctcctggtgctcctgatcgggggcatccccattgcgatgccaacggttctgagcgtgacaatggccatcggcagccacaagctctcgcagcagggggccattacgaagaggatgacagccatcgaggagatggcggggatggacgtcctgtgctctgataagacaggcactctcaccctgaacaagctgtcagtggacaagaatctcgttgaggtgttctgcaagggcgttgacaaggatcacgtgctcctgctcgcggctcgggcctcccgcaccgagaaccaggacgcgatcgatgctgcgatggtggggatgctcgccgatccaaaggaggctagggccggcattcgggagatccatttcctgcccttcaatccagtcgacaagaggactgctctcacctacatcgacgccgatggccactggcatcgggtgagcaagggggccccagagcagatcctcgacctgtgccactgcaaggaggatctgcggcgcaaggtgcatggcatcattgacaagtacgcggagagggggctcaggtcgctggcggtcgctcggcaggaggttcccgagcgcaacaaggagtctcctgggggcccgtggcagttcgtcggcctgctcccactcttcgacccacctcggcacgattccgcggagactatccgcaaggctctcgtgctgggcgtcaatgttaagatgattaccggggatcagctggccatcggcaaggagacggggaggaggctcgggatgggcacaaacatgtacccgtcttcagcgctgctcggccagaataaggacgctaccctggaggccctcccggtggacgagctgatcgagaaggcggatggcttcgctggggtcttcccggagcacaagtacgagattgttaagaggctgcaggagaagaagcatatcgtgggcatgacgggggacggcgtcaacgatgctcctgctctcaagaaggcggatatcggcattgctgtcgctgacgctacggatgctgctcggtcggcctctgacatcgttctgacagagccgggcctctctgtgatcatttcagcggtcctgacctcacgctgcattttccagaggatgaagaactacactatctacgcggtttccatcaccattcgcatcgtgctcggcttcatgctcattgccctgatctggcagtacgacttctctccgttcatggtcctgatcattgccatcctcaatgacggcacgattatgacaatctcaaaggatagggtgaagccatcgcctctgccggactcttggaagctcaaggagattttcgccacaggcatcgtgctggggtcctacctcgctctgatgactgtcatcttcttctgggccatgcacaagaccgacttcttcagcgataagttcggcgtccgctccatcagggacagcgagcatgagatgatgtcggcgctctacctgcaggtctcaattgtttcccaggccctcatcttcgtgacccggtcacgctcctggagcttcgttgagaggccaggcctgctcctggtgacggccttcctcctggcgcagctggtcgctacattcctcgccgtttacgcgaactggggcttcgcgcgcattaaggggatcggctgggggtgggctggcgtcgtttggctgtactccatcgtcttctacttcccgctcgacctgattaagttcttcatcaggttcgtgctcagcggccgggcgtgggataacctcctggagaataagacggccttcaccacgaagaaggactacggcagggaggagcgcgaggctcagctcgctactgctcagcgcaccctccacggcctgcagccaccagaggctgctacgtcgacactgttccatgacaagaactcatacagggagctctccgagattgctgagcaggccaagcgcagggcggagatcgctaggctcagggagctgaacaccctcaaggggcacgtcgagtccgtggtcaagctgaagggcctcgacattgatactatccagcagaattacaccgtgtagaacctaaatgctcttaactgagctaattatgtaatgcacatacacatatttacatagatatgcatatttatatatagcatgtatattgtactacatgcattgcttcttaatacatgtagtaaagatatatgcaaaaatagtcgaaagatttgtttacatataaaatcaccaatatttattgttattgtattttcatgaataaagtaataagattatttgtctaatattttgatttactagtactagaaatgaaaaggaatatgcacaatttcagcattatagtttggtaggcaaaatggagtgagaatagagtttcatagtatatactaaggttcttaattgtgcaaatagttgatacaagtcacatgggccaagtttgtaaatcttaaatcgaaatatgccttcttctttttttgcatgaaaatgctagtaatttataagtgtgtttttcaataagagatgctaaataccaaaattaacctagttttcagtgagcgcttgcattattgtgg

SEQ ID NO: 59 - DNA, 4402 bp, Artificial
  Cassette_T02784_rbcS_Mut_al ZmAHA5_W885L
tccctttaatctggcgctagatctgcatccgcggcttgcaaagataaatggcacatttagtgtgttattttgcaatacctttcatagtagatatccttaaatgcagttttaggcatgtttgggtaattaaataacatttttaggaggagttttagatttacctttctttcgtgatgactgatgacagacgtggggaattcaaatgcaactctagcgaaagttcatatatttttcataaatagctgaggctggggtaattattttttttgtagaaaaatagaataggtggaatggttggggaaggcgtaggcgctcgtggacgacgcccgataaaagacaagaggcggaattgccatgaattcgaggtagctaagtaaggcgcatatatatgccaaaaaattctactgtcactttccaatttcaatgcgctgccaaacaagccatcctggaaactgacttgaattcagcccaattctgtagatccaaacagggccggcgtcagtgcctcaggtgagagagcagcagacgattcaaagagccaaaactgcaagcagacgcagccgaagccgaagccgaagcccaagcccaaaactgttttgtctttgcccagaaccgcgacgagcctaaactgcgcttcctcctatctacaagtccctggcacatcacgcatagtccaacctaggcgcgcaggcgataaggcgcgccacggggacgcgacatgtggtggcggacgcgatcaggatagggccaggctggccgggcgcggccacgggagaacggtggccactcgtcccacatccgcttcgtcctgtcctgtactgcgtcctgcccccaacgagagccggagccggccatcccgtcgcacactctccccctctatatatgccgtcggtgtgggggagcctactacaggacgacccaagcaagcaagcaagcagcgagtacatacatactaggcagccaggcagtctccaccatggggccactgcagcggcggcctacggctatgggggggctggaggagattaagaacgaggcggttgacctggagaacatcccgattgaggaggtgttcgagcagctgaagtgcacccgcgagggcctctccagctcggaggggcagcagcgcctggagatcttcggccccaaccgcctggaggagaagaaggagtccaagatcctcaagttcctgggcttcatgtggaacccactgagctgggttatggagatggctgccgtgatggctatcgcgctcgctaatggcgggggcaagccaccagactgggaggatttcgtcggcatcattgtgctcctggtcatcaactcgacgatttctttcatcgaggagaacaatgctggcaacgctgccgcggctctgatggctaatctcgctcctaagacaaaggtgctgagggatggccgctggggggagcaggaggccgcgatcctggtgccgggcgacattgtcagcatcaagctcggggacatcgttccagctgatgctaggctcctggagggggacccactcaaggtggatcagagcgctctgacgggcgagtcgctccctgtcacaaaggggccaggcgacgaggttttctccggcagcacgtgcaagcagggggagattgaggccgtggtcatcgcgactggcgtccacaccttcttcgggaaggctgcccatctggtcgactcgactaaccaggttggccacttccagcaggtgctcaccgcgatcgggaatttctgcatttgctctatcgctgtgggcattgttgtggagatcattgtcatgttcccaatccagcataggcgctaccgctccggcattgagaacctcctggtgctcctgatcgggggcatccccattgcgatgccaacggttctgagcgtgacaatggccatcggcagccacaagctctcgcagcagggggccattacgaagaggatgacagccatcgaggagatggcggggatggacgtcctgtgctctgataagacaggcactctcaccctgaacaagctgtcagtggacaagaatctcgttgaggtgttctgcaagggcgttgacaaggatcacgtgctcctgctcgcggctcgggcctcccgcaccgagaaccaggacgcgatcgatgctgcgatggtggggatgctcgccgatccaaaggaggctagggccggcattcgggagatccatttcctgcccttcaatccagtcgacaagaggactgctctcacctacatcgacgccgatggccactggcatcgggtgagcaagggggccccagagcagatcctcgacctgtgccactgcaaggaggatctgcggcgcaaggtgcatggcatcattgacaagtacgcggagagggggctcaggtcgctggcggtcgctcggcaggaggttcccgagcgcaacaaggagtctcctgggggcccgtggcagttcgtcggcctgctcccactcttcgacccacctcggcacgattccgcggagactatccgcaaggctctcgtgctgggcgtcaatgttaagatgattaccggggatcagctggccatcggcaaggagacggggaggaggctcgggatgggcacaaacatgtacccgtcttcagcgctgctcggccagaataaggacgctaccctggaggccctcccggtggacgagctgatcgagaaggcggatggcttcgctggggtcttcccggagcacaagtacgagattgttaagaggctgcaggagaagaagcatatcgtgggcatgacgggggacggcgtcaacgatgctcctgctctcaagaaggcggatatcggcattgctgtcgctgacgctacggatgctgctcggtcggcctctgacatcgttctgacagagccgggcctctctgtgatcatttcagcggtcctgacctcacgctgcattttccagaggatgaagaactacactatctacgcggtttccatcaccattcgcatcgtgctcggcttcatgctcattgccctgatctggcagtacgacttctctccgttcatggtcctgatcattgccatcctcaatgacggcacgattatgacaatctcaaaggatagggtgaagccatcgcctctgccggactcttggaagctcaaggagattttcgccacaggcatcgtgctggggtcctacctcgctctgatgactgtcatcttcttctgggccatgcacaagaccgacttcttcagcgataagttcggcgtccgctccatcagggacagcgagcatgagatgatgtcggcgctctacctgcaggtctcaattgtttcccaggccctcatcttcgtgacccggtcacgctcctggagcttcgttgagaggccaggcctgctcctggtgacggccttcctcctggcgcagctggtcgctacattcctcgccgtttacgcgaactggggcttcgcgcgcattaaggggatcggctgggggtgggctggcgtcgtttggctgtactccatcgtcttctacttcccgctcgacctgattaagttcttcatcaggttcgtgctcagcggccgggcgtgggataacctcctggagaataagacggccttcaccacgaagaaggactacggcagggaggagcgcgaggctcagctcgctactgctcagcgcaccctccacggcctgcagccaccagaggctgctacgtcgacactgttccatgacaagaactcatacagggagctctccgagattgctgagcaggccaagcgcagggcggagatcgctaggctcagggagctgaacaccctcaaggggcacgtcgagtccgtggtcaagctgaagggcctcgacattgatactatccagcagaattacaccgtgtagaactagaccgcgcccgccggccgccccccgccggctagctagctagctagctagctcctgcgtgagctagtagctagtgccatgcgtcgtctctgtcgttcggttttgcttcgggtcaccgtaccctttgcttgcttggtttcttctttccttttttccttttttttttcttcttttccccggccatggttcctttgctttcagcagttctctgctggatgtgatgtatccattgttgcaagcatggccttgcattggctacctctatacctgctacaaactactgcaacgcctatatatacttggggtgaggaacatgtgaatgcaagctccggctatcatatacatgtaatatggatacaaactatatatataaatccgccgaggcgccgactaatactatacgacgacaccgtgttaagttaatatataactggtgctttttatttatatatctgtctcatcatatatatatgctaattaatggatgtgtgtcctcttcacttcaattccttctttcctttcctatgctttgagatc

SEQ ID NO: 60 - DNA, 3841 bp, Artificial
  Cassette_T10401_RAB17_del ZmAHA5_W885L
aaatgttatgcagttcgctctggacttttctgctgcgcctacacttgggtgtactgggcctaaattcagcctgaccgaccgcctgcattgaataatggatgagcaccggtaaaatccgcgtacccaactttcgagaagaaccgagacgtggcgggccgggccaccgacgcacggcaccagcgactgcacacgtcccgccggcgtacgtgtacgtgctgttccctcactggccgcccaatccactcatgcatgcccacgtacacccctgccgtggcgcgcccagatcctaatcctttcgccgttctgcacttctgctgcctataaatggcggcatcgaccgtcacctgcttcaccaccggcgagccacatcgagaacacgatcgagcacacaagcacgaagactcgtttaggagaaaccacaaaccaccaagccgtgcaagcatctctccaccatgggcccactgcagaggcgcccaacagcgatggggggcctggaggagatcaagaacgaggccgtcgatctggagaacatccctattgaggaggtgttcgagcagctgaagtgcacccgggagggcctcagctcctcggagggccagcagcgcctggagatcttcggcccaaaccggctggaggagaagaaggagagcaagatcctcaagttcctggggttcatgtggaacccgctgtcctgggtcatggagatggctgccgtgatggcgattgctctggctaatggcgggggcaagccaccggactgggaggatttcgtggggattatcgtcctgctcgtcatcaacagcactatctccttcattgaggagaacaacgctggcaacgccgctgctgcgctgatggcgaacctcgctccaaagactaaggtcctccgcgacggccgctggggggagcaggaggctgcgattctcgtgcccggggacatcgttagcattaagctcggggatatcgtccctgctgatgcccggctgctggagggggaccccctgaaggtcgaccagagcgctctcaccggcgagtcgctcccagtcactaagggccctggggacgaggtgttcagcggctctacgtgcaagcagggcgagatcgaggcggtcgtgatcgctaccggcgtgcacaccttcttcgggaaggccgcccatctcgtggattcgacaaaccaggtcgggcacttccagcaggtgctgacagccatcgggaacttctgcatctgctcgattgccgttgggatcgtggttgagattattgtgatgttcccgattcagcaccggcgctaccgctccgggatcgagaacctcctggtcctcctcattggggggattccgatcgctatgccgaccgtcctgagcgtcactatggctatcgggtctcacaagctctcacagcagggggcgattaccaagcggatgacagcgattgaggagatggcggggatggacgtgctgtgctcagacaagaccggcactctgacgctcaacaagctctccgtggacaagaacctcgtcgaggtgttctgcaagggggtggacaaggatcatgtcctgctgctggcggccagggcctcccggacagagaaccaggacgccattgacgccgctatggtggggatgctggccgaccctaaggaggcgagggccggcatccgcgagattcacttcctgccattcaatcccgttgacaagcgcactgcgctgacgtacattgatgcggacgggcactggcacagggtgtccaagggggctccagagcagatcctcgatctgtgccactgcaaggaggatctgcggcgcaaggtgcatgggatcattgacaagtacgcggagagggggctccggagcctggcggtggccaggcaggaggtgccggagcgcaacaaggagtcgccggggggcccttggcagttcgtcgggctgctccctctgttcgatcccccgaggcacgacagcgcggagactatccgcaaggccctcgttctgggggtgaatgtcaagatgattaccggggaccagctggccattgggaaggagacaggccggcgcctcgggatgggcacgaacatgtacccgtcatccgccctgctggggcagaataaggacgccactctggaggccctgccggtcgatgagctcatcgagaaggctgacgggttcgcgggcgtcttccccgagcataagtacgagatcgtgaagcggctgcaggagaagaagcatattgtggggatgactggcgacggggtgaatgatgctcccgccctgaagaaggctgacatcggcattgccgtcgcggacgccacagatgctgcccgctcggcgtccgatatcgttctcacggagcctgggctgagcgttattatctcggcggttctgacaagcaggtgcatcttccagcgcatgaagaactacaccatctacgctgtgtcgatcactatcaggatcgtgctgggcttcatgctgattgcgctcatctggcagtacgacttctcccctttcatggtcctgatcattgctatcctcaacgacggcacaatcatgactatctcgaaggaccgcgtgaagccgagcccactccccgactcttggaagctcaaggagattttcgccactgggatcgttctcgggtcttacctcgctctgatgaccgtgattttcttctgggctatgcacaagaccgacttcttcagcgacaagttcggggttcgctcgattcgcgactcggagcacgagatgatgtctgcgctgtacctccaggtttcaattgtttcacaggcgctcattttcgtgactaggtcacggtcttggtccttcgtcgagaggcctggcctgctcctggtcactgctttcctgctcgcccagctggtggccactttcctcgctgtttacgctaattgggggttcgctaggatcaaggggatcggctgggggtgggcgggcgtggtctggctctactccatcgttttctacttcccactcgacctcatcaagttcttcattcggttcgtgctgtcagggagggcgtgggacaacctcctggagaacaagaccgcgttcaccactaagaaggactacggccgcgaggagagggaggcgcagctggctacagcgcagcgcaccctccacgggctccagcccccagaggctgcgacatctacactcttccacgacaagaattcttaccgcgagctgtcagagattgccgagcaggctaagcgcagggcggagattgctaggctgagggagctcaacacactgaagggccacgtggagtcagtggtcaagctgaagggcctggacatcgatacaattcagcagaactacaccgtttagaacgcggcgcctatacgtggctgtgctgtgctgtctggcgcgtcaaagccgtactcttcagcgttccatagataataagataaacccatgaataagtgtccctaccctttgatcatgtgacagggacagggacagtttcctgtacttgtggggtgaatttgtacgtgtgatacggtaacttggtccgtgtactgtttatgctgctacgtttccttcctaaaagtacgtatatatatacagcacttgcgagtggctttacttgtgtgcactgcctaaaagtgtcgatattacctccagcggtaaataaatgacccttgtaagaaacttacacagcatgtcttactaattaacagccgttattatgttcggcgcagtactcacactggaacttacgaacaagaattgctctatcaatcaccatctactttagatatatcttctgaaacttttttcaaatccaaaagttcagtatcttcctacaaattagtgaattaggaatccaa

SEQ ID NO: 61 - DNA, 4328 bp, Artificial
  Cassette_T10584_MYB60 ZmAHA5_W885L
ctccgtcgctagcgttgtaatttttatcagcctctctccatctgattggatgagctgcttctcctagctagcacgttgtcaaccattggggacgccctttaggagtgaaagtgatgcagttactctactcccatccggtccaaatcccaacctaagggatatatgacgaagagttttcaatttcagtataatgtgtatagcaagtgatttgattttcctgcagattcttgagagagaagggccaaacctgcatatgtgccaggtgcgcactcacagtcacacacacggtcctcatcaatgcccaagaaatctggagagacacagacaaacgcaagcaattactccattcatgagcgccacagcagaaaaaggagtcctccagaaccggccgtgttcttggcttgcacacacacacacacacacgcgaaagcagcgcatgcaacaaagcaaagatcacacacggccggagcaagagagacgcccatattcatgtgatcacctggctgacttttgcattggaaagcaacagtgcgagatcaaaagcgaacgcagcacacagcacagcacagcacagggatcgagttgctctactccgtatatgaggtcatgcagtatataagcactcacatgcagctataccttagctagggcacctgtgcaaggggacaggtaggagataaagcaatgtctgctggctagaataaaaggaggccgatatcgtatcagcagagggttccaggggagaaggccgttctgcagggccgccgtaaaaggctgtgtaggaagcagccacagcttctcatatcttcttgttcttcgactacttgcctagctactatatctactagactagccctaggctgcttgctagctagtaggtgtatcgatcgtccgaggtaggaggagacagcaggaagcaggctctccaccatgggcccactgcagaggcgcccaacagcgatggggggcctggaggagatcaagaacgaggccgtcgatctggagaacatccctattgaggaggtgttcgagcagctgaagtgcacccgggagggcctcagctcctcggagggccagcagcgcctggagatcttcggcccaaaccggctggaggagaagaaggagagcaagatcctcaagttcctggggttcatgtggaacccgctgtcctgggtcatggagatggctgccgtgatggcgattgctctggctaatggcgggggcaagccaccggactgggaggatttcgtggggattatcgtcctgctcgtcatcaacagcactatctccttcattgaggagaacaacgctggcaacgccgctgctgcgctgatggcgaacctcgctccaaagactaaggtcctccgcgacggccgctggggggagcaggaggctgcgattctcgtgcccggggacatcgttagcattaagctcggggatatcgtccctgctgatgcccggctgctggagggggaccccctgaaggtcgaccagagcgctctcaccggcgagtcgctcccagtcactaagggccctggggacgaggtgttcagcggctctacgtgcaagcagggcgagatcgaggcggtcgtgatcgctaccggcgtgcacaccttcttcgggaaggccgcccatctcgtggattcgacaaaccaggtcgggcacttccagcaggtgctgacagccatcgggaacttctgcatctgctcgattgccgttgggatcgtggttgagattattgtgatgttcccgattcagcaccggcgctaccgctccgggatcgagaacctcctggtcctcctcattggggggattccgatcgctatgccgaccgtcctgagcgtcactatggctatcgggtctcacaagctctcacagcagggggcgattaccaagcggatgacagcgattgaggagatggcggggatggacgtgctgtgctcagacaagaccggcactctgacgctcaacaagctctccgtggacaagaacctcgtcgaggtgttctgcaagggggtggacaaggatcatgtcctgctgctggcggccagggcctcccggacagagaaccaggacgccattgacgccgctatggtggggatgctggccgaccctaaggaggcgagggccggcatccgcgagattcacttcctgccattcaatcccgttgacaagcgcactgcgctgacgtacattgatgcggacgggcactggcacagggtgtccaagggggctccagagcagatcctcgatctgtgccactgcaaggaggatctgcggcgcaaggtgcatgggatcattgacaagtacgcggagagggggctccggagcctggcggtggccaggcaggaggtgccggagcgcaacaaggagtcgccggggggcccttggcagttcgtcgggctgctccctctgttcgatcccccgaggcacgacagcgcggagactatccgcaaggccctcgttctgggggtgaatgtcaagatgattaccggggaccagctggccattgggaaggagacaggccggcgcctcgggatgggcacgaacatgtacccgtcatccgccctgctggggcagaataaggacgccactctggaggccctgccggtcgatgagctcatcgagaaggctgacgggttcgcgggcgtcttccccgagcataagtacgagatcgtgaagcggctgcaggagaagaagcatattgtggggatgactggcgacggggtgaatgatgctcccgccctgaagaaggctgacatcggcattgccgtcgcggacgccacagatgctgcccgctcggcgtccgatatcgttctcacggagcctgggctgagcgttattatctcggcggttctgacaagcaggtgcatcttccagcgcatgaagaactacaccatctacgctgtgtcgatcactatcaggatcgtgctgggcttcatgctgattgcgctcatctggcagtacgacttctcccctttcatggtcctgatcattgctatcctcaacgacggcacaatcatgactatctcgaaggaccgcgtgaagccgagcccactccccgactcttggaagctcaaggagattttcgccactgggatcgttctcgggtcttacctcgctctgatgaccgtgattttcttctgggctatgcacaagaccgacttcttcagcgacaagttcggggttcgctcgattcgcgactcggagcacgagatgatgtctgcgctgtacctccaggtttcaattgtttcacaggcgctcattttcgtgactaggtcacggtcttggtccttcgtcgagaggcctggcctgctcctggtcactgctttcctgctcgcccagctggtggccactttcctcgctgtttacgctaattgggggttcgctaggatcaaggggatcggctgggggtgggcgggcgtggtctggctctactccatcgttttctacttcccactcgacctcatcaagttcttcattcggttcgtgctgtcagggagggcgtgggacaacctcctggagaacaagaccgcgttcaccactaagaaggactacggccgcgaggagagggaggcgcagctggctacagcgcagcgcaccctccacgggctccagcccccagaggctgcgacatctacactcttccacgacaagaattcttaccgcgagctgtcagagattgccgagcaggctaagcgcagggcggagattgctaggctgagggagctcaacacactgaagggccacgtggagtcagtggtcaagctgaagggcctggacatcgatacaattcagcagaactacaccgtttagaacctaaatgctcttaactgagctaattatgtaatgcacatacacatatttacatagatatgcatatttatatatagcatgtatattgtactacatgcattgcttcttaatacatgtagtaaagatatatgcaaaaatagtcgaaagatttgtttacatataaaatcaccaatatttattgttattgtattttcatgaataaagtaataagattatttgtctaatattttgatttactagtactagaaatgaaaaggaatatgcacaatttcagcattatagtttggtaggcaaaatggagtgagaatagagtttcatagtatatactaaggttcttaattgtgcaaatagttgatacaagtcacatgggccaagtttgtaaatcttaaatcgaaatatgccttcttctttttttgcatgaaaatgctagtaatttataagtgtgtttttcaataagagatgctaaataccaaaattaacctagttttcagtgagcgcttgcattattgtgg

SEQ ID NO: 62 - DNA, 2796 bp, Arabidopsis thaliana
  misc_feature: AtAHA5W857L
atggaggaggttttcgaggagctgaagtgcaccaagcaggggctgaccgctaatgaggcgtcccacaggctggatgttttcgggccaaacaagctggaggagaagaaggagtctaagctcctgaagttcctgggcttcatgtggaaccccctctcatgggttatggaggtggctgctctgatggctatcgctctcgccaatggcgggggcaggccgcccgactggcaggatttcgtcggcattgtttgcctcctgctcatcaactctacgatttcattcatcgaggagaacaatgctggcaatgctgccgcggctctgatggccgggctcgcgccaaagacaaaggtgctcagggacaaccagtggtctgagcaggaggcgtcaatcctggtgccaggcgatgtcatctccattaagctcggggacatcattccagctgatgctaggctgctcgacggcgatccactgaagatcgaccagtccagcctcacgggcgagtcgattcccgtcacaaagaacccatctgatgaggttttcagcggctcgatttgcaagcagggggagatcgaggccatcgtcattgcgactggcgttcacaccttcttcgggaaggccgcgcatctggtggacaacactaatcagatcggccacttccagaaggtcctgacctcaattgggaacttctgcatttgctccatcgccctcggcatcattgttgagctgctcgtgatgtacccaatccagaggaggcgctaccgcgacggcattgataatctgctcgtgctgctcatcgggggcatccctattgcgatgccgtccgtgctgagcgtcacgatggctacaggctcccaccgcctcttccagcagggggctattacgaagcgcatgacagctatcgaggagatggccgggatggacgtgctctgctgcgataagacaggcactctgaccctcaacaagctgaccgtcgacaagaatctcgtcgaggttttcgcgaagggggtgggcaaggagcatgtcttcctgctcgctgcccgcgcctcccgcatcgagaaccaggacgccattgatgctgctatcgtcggcatgctggccgacccaaaggaggccagggcgggcgttcgggaggtgcacttcttccctttcaacccggtggacaagcgcactgcgctcacctacgtcgacagcgatggcaattggcatagggcttcgaagggggccccagagcagatcctgaacctctgcaattgcaaggaggacgtgcgcaggaaggtccacggcgttatcgataagttcgctgagagggggctgaggtcgctcgctgttgcccggcaggaggtgctggagaagaagaaggacgctccagggggcccgtggcagctggtcggcctgctccctctcttcgacccacctcgccatgatagcgctgagacgatccggcgcgctctgaacctcggcgtgaatgtcaagatgattacaggggaccagctggccatcggcaaggagacggggaggaggctcgggatgggcacaaacatgtacccgtcgtctgctctgctcggccaggtcaaggactcatccctgggggcgctccctgttgacgagctcatcgagaaggcggatggcttcgctggggttttcccggagcacaagtacgagatcgtgcatcgcctgcagcagaggaaccacatctgcggcatgacgggggacggcgtgaatgatgcgcctgctctcaagaaggccgacatcggcattgccgtggtcgacgctacggatgctgcgaggggggcgagcgatatcgtcctgacagagccgggcctctcagtcatcatttccgccgttctgacctcccgggcgattttccagcgcatgaagaactacactatctacgccgttagcatcaccattcgcatcgtgttcggcttcatgttcattgcgctcatctggcagttcgacttctcgccgttcatggtgctgatcattgccatcctcaatgacggcacgattatgacaatctctaaggataggatgaagccgtccccacagccagacagctggaagctgagggatatcttctccactggcgttgtgctggggggctaccaggctctcatgaccgtcgtgttcttctgggtcatgaaggacagcgacttcttctccaactacttcggcgtcaggcctctgagccagaggccagagcagatgatggctgctctgtacctccaggtgtcgatcatttctcaggccctcatcttcgtcacccggtctcgctcatggtcctacgctgagtgcccaggcctgctcctgctcggggctttcgtgattgcccagctggtcgcgaccttcatcgctgtgtacgccaactggtcattcgcgaggatcgagggggctggctgggggtgggctggcgtcatttggctgtactccttcctcacctacatcccactcgacctgctcaagttcggcattcgctacgtgctgagcgggaaggcctggctcaacctcctggagaataagactgcgttcaccacgaagaaggactacggcaaggaggagcgcgaggctcagctggcggctgcccagaggaccctgcacggcctccagccggcggagaagaacaatatcttcaacgagaagaatagctactcggagctctcgcagatcgctgagcaggctaagcgcagggccgaggtggtcaggctgagggagatcaacacgctcaagggccacgtggagtctgttgtgaagctgaagggcctcgacattgatactatccagcagcattacaccgtctag

SEQ ID NO: 63 - DNA, 4326 bp, Artificial
  Cassette_T02780_CsVMV AtAHA5_W857L
aaggtaattatccaagatgtagcatcaagaatccaatgtttacgggaaaaactatggaagtattatgtgagctcagcaagaagcagatcaatatgcggcacatatgcaacctatgttcaaaaatgaagaatgtacagatacaagatcctatactgccagaatacgaagaagaatacgtagaaattgaaaaagaagaaccaggcgaagaaaagaatcttgaagacgtaagcactgacgacaacaatgaaaagaagaagataaggtcggtgattgtgaaagagacatagaggacacatgtaaggtggaaaatgtaagggcggaaagtaaccttatcacaaaggaatcttatcccccactacttatccttttatatttttccgtgtcatttttgcccttgagttttcctatataaggaaccaagttcggcatttgtgaaaacaagaaaaaatttggtgtaagctattttctttgaagtactgaggatacaacttcagagaaatttgtccctcccccctccccctccgccgccgccgcgccggtaaccaccccgcccctctcctctttctttctccgttttttttttccgtctcggtctcgatctttggccttggtagtttgggtgggcgagaggcggcttcgtgcgcgcccagatcggtgcgcgggaggggcgggatctcgcggctggggctctcgccggcgtggatccggcccggatctcgcggggaatggggctctcggatgtagatctgcgatccgccgttgttgggggagatgatggggggtttaaaatttccgccatgctaaacaagatcaggaagaggggaaaagggcactatggtttatatttttatatatttctgctgcttcgtcaggcttagatgtgctagatctttctttcttctttttgtgggtagaatttgaatccctcagcattgttcatcggtagtttttcttttcatgatttgtgacaaatgcagcctcgtgcggagcttttttgtaggtagacgatatctccaccatggaggaggttttcgaggagctgaagtgcaccaagcaggggctgaccgctaatgaggcgtcccacaggctggatgttttcgggccaaacaagctggaggagaagaaggagtctaagctcctgaagttcctgggcttcatgtggaaccccctctcatgggttatggaggtggctgctctgatggctatcgctctcgccaatggcgggggcaggccgcccgactggcaggatttcgtcggcattgtttgcctcctgctcatcaactctacgatttcattcatcgaggagaacaatgctggcaatgctgccgcggctctgatggccgggctcgcgccaaagacaaaggtgctcagggacaaccagtggtctgagcaggaggcgtcaatcctggtgccaggcgatgtcatctccattaagctcggggacatcattccagctgatgctaggctgctcgacggcgatccactgaagatcgaccagtccagcctcacgggcgagtcgattcccgtcacaaagaacccatctgatgaggttttcagcggctcgatttgcaagcagggggagatcgaggccatcgtcattgcgactggcgttcacaccttcttcgggaaggccgcgcatctggtggacaacactaatcagatcggccacttccagaaggtcctgacctcaattgggaacttctgcatttgctccatcgccctcggcatcattgttgagctgctcgtgatgtacccaatccagaggaggcgctaccgcgacggcattgataatctgctcgtgctgctcatcgggggcatccctattgcgatgccgtccgtgctgagcgtcacgatggctacaggctcccaccgcctcttccagcagggggctattacgaagcgcatgacagctatcgaggagatggccgggatggacgtgctctgctgcgataagacaggcactctgaccctcaacaagctgaccgtcgacaagaatctcgtcgaggttttcgcgaagggggtgggcaaggagcatgtcttcctgctcgctgcccgcgcctcccgcatcgagaaccaggacgccattgatgctgctatcgtcggcatgctggccgacccaaaggaggccagggcgggcgttcgggaggtgcacttcttccctttcaacccggtggacaagcgcactgcgctcacctacgtcgacagcgatggcaattggcatagggcttcgaagggggccccagagcagatcctgaacctctgcaattgcaaggaggacgtgcgcaggaaggtccacggcgttatcgataagttcgctgagagggggctgaggtcgctcgctgttgcccggcaggaggtgctggagaagaagaaggacgctccagggggcccgtggcagctggtcggcctgctccctctcttcgacccacctcgccatgatagcgctgagacgatccggcgcgctctgaacctcggcgtgaatgtcaagatgattacaggggaccagctggccatcggcaaggagacggggaggaggctcgggatgggcacaaacatgtacccgtcgtctgctctgctcggccaggtcaaggactcatccctgggggcgctccctgttgacgagctcatcgagaaggcggatggcttcgctggggttttcccggagcacaagtacgagatcgtgcatcgcctgcagcagaggaaccacatctgcggcatgacgggggacggcgtgaatgatgcgcctgctctcaagaaggccgacatcggcattgccgtggtcgacgctacggatgctgcgaggggggcgagcgatatcgtcctgacagagccgggcctctcagtcatcatttccgccgttctgacctcccgggcgattttccagcgcatgaagaactacactatctacgccgttagcatcaccattcgcatcgtgttcggcttcatgttcattgcgctcatctggcagttcgacttctcgccgttcatggtgctgatcattgccatcctcaatgacggcacgattatgacaatctctaaggataggatgaagccgtccccacagccagacagctggaagctgagggatatcttctccactggcgttgtgctggggggctaccaggctctcatgaccgtcgtgttcttctgggtcatgaaggacagcgacttcttctccaactacttcggcgtcaggcctctgagccagaggccagagcagatgatggctgctctgtacctccaggtgtcgatcatttctcaggccctcatcttcgtcacccggtctcgctcatggtcctacgctgagtgcccaggcctgctcctgctcggggctttcgtgattgcccagctggtcgcgaccttcatcgctgtgtacgccaactggtcattcgcgaggatcgagggggctggctgggggtgggctggcgtcatttggctgtactccttcctcacctacatcccactcgacctgctcaagttcggcattcgctacgtgctgagcgggaaggcctggctcaacctcctggagaataagactgcgttcaccacgaagaaggactacggcaaggaggagcgcgaggctcagctggcggctgcccagaggaccctgcacggcctccagccggcggagaagaacaatatcttcaacgagaagaatagctactcggagctctcgcagatcgctgagcaggctaagcgcagggccgaggtggtcaggctgagggagatcaacacgctcaagggccacgtggagtctgttgtgaagctgaagggcctcgacattgatactatccagcagcattacaccgtctagaacctaaatgctcttaactgagctaattatgtaatgcacatacacatatttacatagatatgcatatttatatatagcatgtatattgtactacatgcattgcttcttaatacatgtagtaaagatatatgcaaaaatagtcgaaagatttgtttacatataaaatcaccaatatttattgttattgtattttcatgaataaagtaataagattatttgtctaatattttgatttactagtactagaaatgaaaaggaatatgcacaatttcagcattatagtttggtaggcaaaatggagtgagaatagagtttcatagtatatactaaggttcttaattgtgcaaatagttgatacaagtcacatgggccaagtttgtaaatcttaaatcgaaatatgccttcttctttttttgcatgaaaatgctagtaatttataagtgtgtttttcaataagagatgctaaataccaaaattaacctagttttcagtgagcgcttgcattattgtgg

SEQ ID NO: 64 - DNA, 4312 bp, Artificial
  Cassette_T02783_rbcS_Mut_al AtAHA5_W857L
tccctttaatctggcgctagatctgcatccgcggcttgcaaagataaatggcacatttagtgtgttattttgcaatacctttcatagtagatatccttaaatgcagttttaggcatgtttgggtaattaaataacatttttaggaggagttttagatttacctttctttcgtgatgactgatgacagacgtggggaattcaaatgcaactctagcgaaagttcatatatttttcataaatagctgaggctggggtaattattttttttgtagaaaaatagaataggtggaatggttggggaaggcgtaggcgctcgtggacgacgcccgataaaagacaagaggcggaattgccatgaattcgaggtagctaagtaaggcgcatatatatgccaaaaaattctactgtcactttccaatttcaatgcgctgccaaacaagccatcctggaaactgacttgaattcagcccaattctgtagatccaaacagggccggcgtcagtgcctcaggtgagagagcagcagacgattcaaagagccaaaactgcaagcagacgcagccgaagccgaagccgaagcccaagcccaaaactgttttgtctttgcccagaaccgcgacgagcctaaactgcgcttcctcctatctacaagtccctggcacatcacgcatagtccaacctaggcgcgcaggcgataaggcgcgccacggggacgcgacatgtggtggcggacgcgatcaggatagggccaggctggccgggcgcggccacgggagaacggtggccactcgtcccacatccgcttcgtcctgtcctgtactgcgtcctgcccccaacgagagccggagccggccatcccgtcgcacactctccccctctatatatgccgtcggtgtgggggagcctactacaggacgacccaagcaagcaagcaagcagcgagtacatacatactaggcagccaggcagtctccaccatggaggaggttttcgaggagctgaagtgcaccaagcaggggctgaccgctaatgaggcgtcccacaggctggatgttttcgggccaaacaagctggaggagaagaaggagtctaagctcctgaagttcctgggcttcatgtggaaccccctctcatgggttatggaggtggctgctctgatggctatcgctctcgccaatggcgggggcaggccgcccgactggcaggatttcgtcggcattgtttgcctcctgctcatcaactctacgatttcattcatcgaggagaacaatgctggcaatgctgccgcggctctgatggccgggctcgcgccaaagacaaaggtgctcagggacaaccagtggtctgagcaggaggcgtcaatcctggtgccaggcgatgtcatctccattaagctcggggacatcattccagctgatgctaggctgctcgacggcgatccactgaagatcgaccagtccagcctcacgggcgagtcgattcccgtcacaaagaacccatctgatgaggttttcagcggctcgatttgcaagcagggggagatcgaggccatcgtcattgcgactggcgttcacaccttcttcgggaaggccgcgcatctggtggacaacactaatcagatcggccacttccagaaggtcctgacctcaattgggaacttctgcatttgctccatcgccctcggcatcattgttgagctgctcgtgatgtacccaatccagaggaggcgctaccgcgacggcattgataatctgctcgtgctgctcatcgggggcatccctattgcgatgccgtccgtgctgagcgtcacgatggctacaggctcccaccgcctcttccagcagggggctattacgaagcgcatgacagctatcgaggagatggccgggatggacgtgctctgctgcgataagacaggcactctgaccctcaacaagctgaccgtcgacaagaatctcgtcgaggttttcgcgaagggggtgggcaaggagcatgtcttcctgctcgctgcccgcgcctcccgcatcgagaaccaggacgccattgatgctgctatcgtcggcatgctggccgacccaaaggaggccagggcgggcgttcgggaggtgcacttcttccctttcaacccggtggacaagcgcactgcgctcacctacgtcgacagcgatggcaattggcatagggcttcgaagggggccccagagcagatcctgaacctctgcaattgcaaggaggacgtgcgcaggaaggtccacggcgttatcgataagttcgctgagagggggctgaggtcgctcgctgttgcccggcaggaggtgctggagaagaagaaggacgctccagggggcccgtggcagctggtcggcctgctccctctcttcgacccacctcgccatgatagcgctgagacgatccggcgcgctctgaacctcggcgtgaatgtcaagatgattacaggggaccagctggccatcggcaaggagacggggaggaggctcgggatgggcacaaacatgtacccgtcgtctgctctgctcggccaggtcaaggactcatccctgggggcgctccctgttgacgagctcatcgagaaggcggatggcttcgctggggttttcccggagcacaagtacgagatcgtgcatcgcctgcagcagaggaaccacatctgcggcatgacgggggacggcgtgaatgatgcgcctgctctcaagaaggccgacatcggcattgccgtggtcgacgctacggatgctgcgaggggggcgagcgatatcgtcctgacagagccgggcctctcagtcatcatttccgccgttctgacctcccgggcgattttccagcgcatgaagaactacactatctacgccgttagcatcaccattcgcatcgtgttcggcttcatgttcattgcgctcatctggcagttcgacttctcgccgttcatggtgctgatcattgccatcctcaatgacggcacgattatgacaatctctaaggataggatgaagccgtccccacagccagacagctggaagctgagggatatcttctccactggcgttgtgctggggggctaccaggctctcatgaccgtcgtgttcttctgggtcatgaaggacagcgacttcttctccaactacttcggcgtcaggcctctgagccagaggccagagcagatgatggctgctctgtacctccaggtgtcgatcatttctcaggccctcatcttcgtcacccggtctcgctcatggtcctacgctgagtgcccaggcctgctcctgctcggggctttcgtgattgcccagctggtcgcgaccttcatcgctgtgtacgccaactggtcattcgcgaggatcgagggggctggctgggggtgggctggcgtcatttggctgtactccttcctcacctacatcccactcgacctgctcaagttcggcattcgctacgtgctgagcgggaaggcctggctcaacctcctggagaataagactgcgttcaccacgaagaaggactacggcaaggaggagcgcgaggctcagctggcggctgcccagaggaccctgcacggcctccagccggcggagaagaacaatatcttcaacgagaagaatagctactcggagctctcgcagatcgctgagcaggctaagcgcagggccgaggtggtcaggctgagggagatcaacacgctcaagggccacgtggagtctgttgtgaagctgaagggcctcgacattgatactatccagcagcattacaccgtctagaactagaccgcgcccgccggccgccccccgccggctagctagctagctagctagctcctgcgtgagctagtagctagtgccatgcgtcgtctctgtcgttcggttttgcttcgggtcaccgtaccctttgcttgcttggtttcttctttccttttttccttttttttttcttcttttccccggccatggttcctttgctttcagcagttctctgctggatgtgatgtatccattgttgcaagcatggccttgcattggctacctctatacctgctacaaactactgcaacgcctatatatacttggggtgaggaacatgtgaatgcaagctccggctatcatatacatgtaatatggatacaaactatatatataaatccgccgaggcgccgactaatactatacgacgacaccgtgttaagttaatatataactggtgctttttatttatatatctgtctcatcatatatatatgctaattaatggatgtgtgtcctcttcacttcaattccttctttcctttcctatgctttgagatc

SEQ ID NO: 65 - DNA, 5181 bp, Artificial
  Cassette_T10191_RAB17_del AtAHA5_W857L
aaatgttatgcagttcgctctggacttttctgctgcgcctacacttgggtgtactgggcctaaattcagcctgaccgaccgcctgcattgaataatggatgagcaccggtaaaatccgcgtacccaactttcgagaagaaccgagacgtggcgggccgggccaccgacgcacggcaccagcgactgcacacgtcccgccggcgtacgtgtacgtgctgttccctcactggccgcccaatccactcatgcatgcccacgtacacccctgccgtggcgcgcccagatcctaatcctttcgccgttctgcacttctgctgcctataaatggcggcatcgaccgtcacctgcttcaccaccggcgagccacatcgagaacacgatcgagcacacaagcacgaagactcgtttaggagaaaccacaaaccaccaagccgtgcaagcatctctccaccatggaggaggttttcgaggagctgaagtgcaccaagcaggggctgaccgctaatgaggcgtcccacaggctggatgttttcgggccaaacaagctggaggagaagaaggagtctaagctcctgaagttcctgggcttcatgtggaaccccctctcatgggttatggaggtggctgctctgatggctatcgctctcgccaatggcgggggcaggccgcccgactggcaggatttcgtcggcattgtttgcctcctgctcatcaactctacgatttcattcatcgaggagaacaatgctggcaatgctgccgcggctctgatggccgggctcgcgccaaagacaaaggtgctcagggacaaccagtggtctgagcaggaggcgtcaatcctggtgccaggcgatgtcatctccattaagctcggggacatcattccagctgatgctaggctgctcgacggcgatccactgaagatcgaccagtccagcctcacgggcgagtcgattcccgtcacaaagaacccatctgatgaggttttcagcggctcgatttgcaagcagggggagatcgaggccatcgtcattgcgactggcgttcacaccttcttcgggaaggccgcgcatctggtggacaacactaatcagatcggccacttccagaaggtcctgacctcaattgggaacttctgcatttgctccatcgccctcggcatcattgttgagctgctcgtgatgtacccaatccagaggaggcgctaccgcgacggcattgataatctgctcgtgctgctcatcgggggcatccctattgcgatgccgtccgtgctgagcgtcacgatggctacaggctcccaccgcctcttccagcagggggctattacgaagcgcatgacagctatcgaggagatggccgggatggacgtgctctgctgcgataagacaggcactctgaccctcaacaagctgaccgtcgacaagaatctcgtcgaggttttcgcgaagggggtgggcaaggagcatgtcttcctgctcgctgcccgcgcctcccgcatcgagaaccaggacgccattgatgctgctatcgtcggcatgctggccgacccaaaggaggccagggcgggcgttcgggaggtgcacttcttccctttcaacccggtggacaagcgcactgcgctcacctacgtcgacagcgatggcaattggcatagggcttcgaagggggccccagagcagatcctgaacctctgcaattgcaaggaggacgtgcgcaggaaggtccacggcgttatcgataagttcgctgagagggggctgaggtcgctcgctgttgcccggcaggaggtgctggagaagaagaaggacgctccagggggcccgtggcagctggtcggcctgctccctctcttcgacccacctcgccatgatagcgctgagacgatccggcgcgctctgaacctcggcgtgaatgtcaagatgattacaggggaccagctggccatcggcaaggagacggggaggaggctcgggatgggcacaaacatgtacccgtcgtctgctctgctcggccaggtcaaggactcatccctgggggcgctccctgttgacgagctcatcgagaaggcggatggcttcgctggggttttcccggagcacaagtacgagatcgtgcatcgcctgcagcagaggaaccacatctgcggcatgacgggggacggcgtgaatgatgcgcctgctctcaagaaggccgacatcggcattgccgtggtcgacgctacggatgctgcgaggggggcgagcgatatcgtcctgacagagccgggcctctcagtcatcatttccgccgttctgacctcccgggcgattttccagcgcatgaagaactacactatctacgccgttagcatcaccattcgcatcgtgttcggcttcatgttcattgcgctcatctggcagttcgacttctcgccgttcatggtgctgatcattgccatcctcaatgacggcacgattatgacaatctctaaggataggatgaagccgtccccacagccagacagctggaagctgagggatatcttctccactggcgttgtgctggggggctaccaggctctcatgaccgtcgtgttcttctgggtcatgaaggacagcgacttcttctccaactacttcggcgtcaggcctctgagccagaggccagagcagatgatggctgctctgtacctccaggtgtcgatcatttctcaggccctcatcttcgtcacccggtctcgctcatggtcctacgctgagtgcccaggcctgctcctgctcggggctttcgtgattgcccagctggtcgcgaccttcatcgctgtgtacgccaactggtcattcgcgaggatcgagggggctggctgggggtgggctggcgtcatttggctgtactccttcctcacctacatcccactcgacctgctcaagttcggcattcgctacgtgctgagcgggaaggcctggctcaacctcctggagaataagactgcgttcaccacgaagaaggactacggcaaggaggagcgcgaggctcagctggcggctgcccagaggaccctgcacggcctccagccggcggagaagaacaatatcttcaacgagaagaatagctactcggagctctcgcagatcgctgagcaggctaagcgcagggccgaggtggtcaggctgagggagatcaacacgctcaagggccacgtggagtctgttgtgaagctgaagggcctcgacattgatactatccagcagcattacaccgtctagaacgcggcgcctatacgtggctgtgctgtgctgtctggcgcgtcaaagccgtactcttcagcgttccatagataataagataaacccatgaataagtgtccctaccctttgatcatgtgacagggacagggacagtttcctgtacttgtggggtgaatttgtacgtgtgatacggtaacttggtccgtgtactgtttatgctgctacgtttccttcctaaaagtacgtatatatatacagcacttgcgagtggctttacttgtgtgcactgcctaaaagtgtcgatattacctccagcggtaaataaatgacccttgtaagaaacttacacagcatgtcttactaattaacagccgttattatgttcggcgcagtactcacactggaacttacgaacaagaattgctctatcaatcaccatctactttagatatatcttctgaaacttttttcaaatccaaaagttcagtatcttcctacaaattagtgaattaggaatccaagtggttaaacgaattcggccggccggtaccccttaggcctagggctagaggacccagctttgagtggccgtagatttgcaaaagcaatggctaacagacacatattctgccaaaccccaagaaggataatcacttttcttagataaaaaagaacagaccaatatacaaacatccacacttctgcaaacaatacatcagaactaggattacgccgattacgtggctttagcagactgtccaaaaatctgttttgcaaagctccaattgctccttgcttatccagcttcttttgtgttggcaaactgcgcttttccaaccgattttgttcttctcgcgctttcttcttagcctaaacaaacctcaccgtgcacgcagccatggtcctgaaccttcacctcgtccctataaaagcctagccaaccttcacaatcttatcatcacccacaacaccgagcaccacaaactagagatcctctccaccatggctcagtcaaagcacgggctcacaaaggagatgactatgaagtacaggatggagggctgcgtcgatgggcacaagttcgttatcaccggcgaggggatcggctacccgttcaagggcaagcaggcgattaacctgtgcgtggtcgagggcgggccactgcccttcgctgaggatatcctctccgccgcgttcatgtacggcaacagggttttcaccgagtacccgcaggacattgtcgattacttcaagaattcctgcccagctgggtacacgtgggacaggagcttcctcttcgaggatggcgctgtgtgcatctgcaacgccgacattaccgtttcggtggaggagaattgcatgtaccacgagtctaagttctacggggtgaacttcccagctgacggccccgtcatgaagaagatgacggataattgggagccatcatgcgagaagatcattccagtgcctaagcaggggatcctgaagggcgacgtctccatgtacctcctgctcaaggatggcggcaggctcaggtgccagttcgacacagtctacaaggccaagagcgttccacgcaagatgcctgactggcacttcatccagcataagctgactcgggaggaccgctcggatgcgaagaaccagaagtggcacctgactgagcacgctatcgcctcggggtccgccctcccttgaaacgatcgttcaaacatttggcaataaagtttcttaagattgaatcctgttgccggtcttgcgatgattatcatataatttctgttgaattacgttaagcatgtaataattaacatgtaatgcatgacgttatttatgagatgggtttttatgattagagtcccgcaattatacatttaatacgcgatagaaaacaaaatatagcgcgcaaactaggataaattatcgcgcgcggtgtcatctatgttactag

SEQ ID NO: 66 - DNA, 4238 bp, Artificial
  Cassette_T10586_MYB60 AtAHA5_W857L
ctccgtcgctagcgttgtaatttttatcagcctctctccatctgattggatgagctgcttctcctagctagcacgttgtcaaccattggggacgccctttaggagtgaaagtgatgcagttactctactcccatccggtccaaatcccaacctaagggatatatgacgaagagttttcaatttcagtataatgtgtatagcaagtgatttgattttcctgcagattcttgagagagaagggccaaacctgcatatgtgccaggtgcgcactcacagtcacacacacggtcctcatcaatgcccaagaaatctggagagacacagacaaacgcaagcaattactccattcatgagcgccacagcagaaaaaggagtcctccagaaccggccgtgttcttggcttgcacacacacacacacacacgcgaaagcagcgcatgcaacaaagcaaagatcacacacggccggagcaagagagacgcccatattcatgtgatcacctggctgacttttgcattggaaagcaacagtgcgagatcaaaagcgaacgcagcacacagcacagcacagcacagggatcgagttgctctactccgtatatgaggtcatgcagtatataagcactcacatgcagctataccttagctagggcacctgtgcaaggggacaggtaggagataaagcaatgtctgctggctagaataaaaggaggccgatatcgtatcagcagagggttccaggggagaaggccgttctgcagggccgccgtaaaaggctgtgtaggaagcagccacagcttctcatatcttcttgttcttcgactacttgcctagctactatatctactagactagccctaggctgcttgctagctagtaggtgtatcgatcgtccgaggtaggaggagacagcaggaagcaggctctccaccatggaggaggttttcgaggagctgaagtgcaccaagcaggggctgaccgctaatgaggcgtcccacaggctggatgttttcgggccaaacaagctggaggagaagaaggagtctaagctcctgaagttcctgggcttcatgtggaaccccctctcatgggttatggaggtggctgctctgatggctatcgctctcgccaatggcgggggcaggccgcccgactggcaggatttcgtcggcattgtttgcctcctgctcatcaactctacgatttcattcatcgaggagaacaatgctggcaatgctgccgcggctctgatggccgggctcgcgccaaagacaaaggtgctcagggacaaccagtggtctgagcaggaggcgtcaatcctggtgccaggcgatgtcatctccattaagctcggggacatcattccagctgatgctaggctgctcgacggcgatccactgaagatcgaccagtccagcctcacgggcgagtcgattcccgtcacaaagaacccatctgatgaggttttcagcggctcgatttgcaagcagggggagatcgaggccatcgtcattgcgactggcgttcacaccttcttcgggaaggccgcgcatctggtggacaacactaatcagatcggccacttccagaaggtcctgacctcaattgggaacttctgcatttgctccatcgccctcggcatcattgttgagctgctcgtgatgtacccaatccagaggaggcgctaccgcgacggcattgataatctgctcgtgctgctcatcgggggcatccctattgcgatgccgtccgtgctgagcgtcacgatggctacaggctcccaccgcctcttccagcagggggctattacgaagcgcatgacagctatcgaggagatggccgggatggacgtgctctgctgcgataagacaggcactctgaccctcaacaagctgaccgtcgacaagaatctcgtcgaggttttcgcgaagggggtgggcaaggagcatgtcttcctgctcgctgcccgcgcctcccgcatcgagaaccaggacgccattgatgctgctatcgtcggcatgctggccgacccaaaggaggccagggcgggcgttcgggaggtgcacttcttccctttcaacccggtggacaagcgcactgcgctcacctacgtcgacagcgatggcaattggcatagggcttcgaagggggccccagagcagatcctgaacctctgcaattgcaaggaggacgtgcgcaggaaggtccacggcgttatcgataagttcgctgagagggggctgaggtcgctcgctgttgcccggcaggaggtgctggagaagaagaaggacgctccagggggcccgtggcagctggtcggcctgctccctctcttcgacccacctcgccatgatagcgctgagacgatccggcgcgctctgaacctcggcgtgaatgtcaagatgattacaggggaccagctggccatcggcaaggagacggggaggaggctcgggatgggcacaaacatgtacccgtcgtctgctctgctcggccaggtcaaggactcatccctgggggcgctccctgttgacgagctcatcgagaaggcggatggcttcgctggggttttcccggagcacaagtacgagatcgtgcatcgcctgcagcagaggaaccacatctgcggcatgacgggggacggcgtgaatgatgcgcctgctctcaagaaggccgacatcggcattgccgtggtcgacgctacggatgctgcgaggggggcgagcgatatcgtcctgacagagccgggcctctcagtcatcatttccgccgttctgacctcccgggcgattttccagcgcatgaagaactacactatctacgccgttagcatcaccattcgcatcgtgttcggcttcatgttcattgcgctcatctggcagttcgacttctcgccgttcatggtgctgatcattgccatcctcaatgacggcacgattatgacaatctctaaggataggatgaagccgtccccacagccagacagctggaagctgagggatatcttctccactggcgttgtgctggggggctaccaggctctcatgaccgtcgtgttcttctgggtcatgaaggacagcgacttcttctccaactacttcggcgtcaggcctctgagccagaggccagagcagatgatggctgctctgtacctccaggtgtcgatcatttctcaggccctcatcttcgtcacccggtctcgctcatggtcctacgctgagtgcccaggcctgctcctgctcggggctttcgtgattgcccagctggtcgcgaccttcatcgctgtgtacgccaactggtcattcgcgaggatcgagggggctggctgggggtgggctggcgtcatttggctgtactccttcctcacctacatcccactcgacctgctcaagttcggcattcgctacgtgctgagcgggaaggcctggctcaacctcctggagaataagactgcgttcaccacgaagaaggactacggcaaggaggagcgcgaggctcagctggcggctgcccagaggaccctgcacggcctccagccggcggagaagaacaatatcttcaacgagaagaatagctactcggagctctcgcagatcgctgagcaggctaagcgcagggccgaggtggtcaggctgagggagatcaacacgctcaagggccacgtggagtctgttgtgaagctgaagggcctcgacattgatactatccagcagcattacaccgtctagaacctaaatgctcttaactgagctaattatgtaatgcacatacacatatttacatagatatgcatatttatatatagcatgtatattgtactacatgcattgcttcttaatacatgtagtaaagatatatgcaaaaatagtcgaaagatttgtttacatataaaatcaccaatatttattgttattgtattttcatgaataaagtaataagattatttgtctaatattttgatttactagtactagaaatgaaaaggaatatgcacaatttcagcattatagtttggtaggcaaaatggagtgagaatagagtttcatagtatatactaaggttcttaattgtgcaaatagttgatacaagtcacatgggccaagtttgtaaatcttaaatcgaaatatgccttcttctttttttgcatgaaaatgctagtaatttataagtgtgtttttcaataagagatgctaaataccaaaattaacctagttttcagtgagcgcttgcattattgtgg